European Patent Specification EP 3 701 043 B1, published November 22, 2023. Title: A NONINVASIVE MOLECULAR CLOCK FOR FETAL DEVELOPMENT PREDICTS GESTATIONAL AGE AND PRETERM DELIVERY-II. Applicant: CHAN ZUCKERBERG BIOHUB, INC. THE BOARD OF TRUSTEES OF THE LELAND STANFORD JUNIOR UNIVERSITY. The sequence listing filed with the application follows.

SEQUENCE LISTING (299 sequences)

SEQ ID NO: 1 - DNA, 861 bp, Homo sapiens
acactctgctggtataaaagcaggtgaggacttcattaactgcagttactgagaactcataagacgaagctaaaatccctcttcggatccacagtcaaccgccctgaacacatcctgcaaaaagcccagagaaaggagcgccatggattactacagaaaatatgcagctatctttctggtcacattgtcggtgtttctgcatgttctccattccgctcctgatgtgcaggagacagggtttcaccatgttgcccaggctgctctcaaactcctgagctcaagcaatccacccactaaggcctcccaaagtgctaggattacagattgcccagaatgcacgctacaggaaaacccattcttctcccagccgggtgccccaatacttcagtgcatgggctgctgcttctctagagcatatcccactccactaaggtccaagaagacgatgttggtccaaaagaacgtcacctcagagtccacttgctgtgtagctaaatcatataacagggtcacagtaatggggggtttcaaagtggagaaccacacggcgtgccactgcagtacttgttattatcacaaatcttaaatgttttaccaagtgctgtcttgatgactgctgattttctggaatggaaaattaagttgtttagtgtttatggctttgtgagataaaactctccttttccttaccataccactttgacacgcttcaaggatatactgcagctttactgccttcctccttatcctacagtacaatcagcagtctagttcttttcatttggaatgaatacagcatttagcttgttccactgcaaataaagccttttaaatcatcattcaaaaaaaaaaaaaaaaaaa

SEQ ID NO: 2 - DNA, 3604 bp, Homo sapiens
gagcagagcttggtacagcccaaatagttttcaggttaagaaagccagaatctttgttcagccacactgactgaacagacttttagtggggttacctggctaacagcagcagcggcaacggcagcagcagcagcagcagcagcagcagcagcagcagggctcctgggataactcaggcatagttcaacactatgggtcctcctctgaagctcttcaaaaaccagaaataccaggaactgaagcaggaatgcatcaaagacagcagacttttctgtgatccaacatttctgcctgagaatgattctcttttctacaaccgactgcttcctggaaaggtggtgtggaaacgtccccaggacatctgtgatgacccccatctgattgtgggcaacattagcaaccaccagctgacccaagggagactggggcacaagccaatggtttctgcattttcctgtttggctgttcaggagtctcattggacaaagacaattcccaaccataaggaacaggaatgggaccctcaaaaaacagaaaaatacgctgggatatttcactttcgtttctggcattttggagaatggactgaagtggtgattgatgacttgttgcccaccattaacggagatctggtcttctctttctccacttccatgaatgagttttggaatgctctgctggaaaaagcttatgcaaagctgctaggctgttatgaggccctggatggtttgaccatcactgatattattgtggacttcacgggcacattggctgaaactgttgacatgcagaaaggaagatacactgagcttgttgaggagaagtacaagctattcggagaactgtacaaaacatttaccaaaggtggtctgatctgctgttccattgagtctcccaatcaggaggagcaagaagttgaaactgattggggtctgctgaagggccatacctataccatgactgatattcgcaaaattcgtcttggagagagacttgtggaagtcttcagtgctgagaaggtgtatatggttcgcctgagaaaccccttgggaagacaggaatggagtggcccctggagtgaaatttctgaagagtggcagcaactgactgcatcagatcgcaagaacctggggcttgttatgtctgatgatggagagttttggatgagcttggaggacttttgccgcaactttcacaaactgaatgtctgccgcaatgtgaacaaccctatttttggccgaaaggagctggaatcggtgttgggatgctggactgtggatgatgatcccctgatgaaccgctcaggaggctgctataacaaccgtgataccttcctgcagaatccccagtacatcttcactgtgcctgaggatgggcacaaggtcattatgtcactgcagcagaaggacctgcgcacttaccgccgaatgggaagacctgacaattacatcattggctttgagctcttcaaggtggagatgaaccgcaaattccgcctccaccacctctacatccaggagcgtgctgggacttccacctatattgacacccgcacagtgtttctgagcaagtacctgaagaagggcaactatgtgcttgtcccaaccatgttccagcatggtcgcaccagcgagtttctcctgagaatcttctctgaagtgcctgtccagctcagggaactgactctggacatgcccaaaatgtcctgctggaacctggctcgtggctacccgaaagtagttactcagatcactgttcacagtgctgaggacctggagaagaagtatgccaatgaaactgtaaacccatatttggtcatcaaatgtggaaaggaggaagtccgttctcctgtccagaagaatacagttcatgccatttttgacacccaggccattttctacagaaggaccactgacattcctattatagtacaggtctggaacagccgaaaattctgtgatcagttcttggggcaggttactctggatgctgaccccagcgactgccgtgatctgaagtctctgtacctgcgtaagaagggtggtccaactgccaaagtcaagcaaggccacatcagcttcaaggttatttccagcgatgatctcactgagctctaaatctgcaatcccagagaatcctgacaaagcgtgccacccttttattttccgtcaggtgccaggtcttagttaagattcacaatctttagaaagaatgagattcacaataattaactcttcctctcttctgataaattccccatacctcccaatccaagtagcatctgtagctacataacctatatacctccagcagctggacatggggaggcgacagtcctatctagacatcatacacatttgccaagaaaggatctctggggcttccgggggtgagattcaagcaggacaataacaagaggctggacaccctacagatgtctttgatgttttcagttgtttgatatatctcccctgtagggcatgttgaggaaggaggagggctgatcaaggccaagctggtctagcctgacatcctagctcctgactgaacactatagacttcccagcagcatttcacccagcagccagagccggctttaagtccccaacccttacagacaccactgccaccaccaccaaccacgaccaccaccaccaccaccactcaccaccatcatcacctccggaaagtgtagtcctgccctaacccaagtcacccccgacagtaaattttaccttcatgttgagaaagcttcctggtgcttaatcaagagctggagttcaatgagtcctagacagtgagaggggcctgagcttcagctcaatggaagcctgctgtgtgccacaagacggaaaagtggaagaagctgcagtgggagacaaagcctcggtcccccacccatccacacacacctacactcacacacgcgcacatgggcgcgcacgaactaccattcaggcagtcagtgggcaagaggaaagataagtaagtaccatacacacctaaaagatgagagaattcatccagacatattacagccagtttggggcccctgactgcaatgtgaaacctctcgctgctgctaggtttacaaacaagcccattgtcctgtgcctcctaatatcatttgtactgaagaccccatctggggacttgagactttggtcccagcccagactcctcagacttttctctcagttgggatgcttcactcgctgggggtgtttgtttgccctctcatttttcagtacttctacagaattttctctagagtcagtcattatgaaatgtacttccctccatcttaacctatcaactttctgcccctccttcaaggcccagtataaatgccacctcctccatgaagccttccctaattccaccccaaacccccaccttcaacaatatttcaacgcttctgcaatgatgaaaaagaaacatagttgtagtacttagcctacctagaccagcaagcattcatttttagctcgctcattttttaccatgttttccagtctgtttaacttctgcagtgccttcactacactgccttacataaaccaaatcacaataaagttcatattcagtacattgaaaaaaaaaa

SEQ ID NO: 3 - DNA, 933 bp, Homo sapiens
tgcaggaaagcctcaagtagaggagggttgaggcttcagtccagcacctttctcgggtcacggcctcctcctggctcccaggaccccaccataggcagaggcaggccttcctacaccctactccctgtgcctccagcctcgactagtccctagcactcgacgactgagtctctgaggtcacttcaccgtggtctccgcctcacccttggcgctggaccagtgagaggagagggctggggcgctccgctgagccactcctgcgcccccctggccttgtctacctcttgccccccgaggggttagtgtcgagctcaccccagcatcctatcacctcctggtggccttgccgcccccacaaccccgaggtataaagccaggtacacgaggcaggggacgcaccaaggatggagatgttccaggggctgctgctgttgctgctgctgagcatgggcgggacatgggcatccaaggagccgcttcggccacggtgccgccccatcaatgccaccctggctgtggagaaggagggctgccccgtgtgcatcaccgtcaacaccaccatctgtgccggctactgccccaccatgacccgcgtgctgcagggggtcctgccggccctgcctcaggtggtgtgcaactaccgcgatgtgcgcttcgagtccatccggctccctggctgcccgcgcggcgtgaaccccgtggtctcctacgccgtggctctcagctgtcaatgtgcactctgccgccgcagcaccactgactgcgggggtcccaaggaccaccccttgacctgtgatgacccccgcttccaggactcctcttcctcaaaggcccctccccccagccttccaagcccatcccgactcccggggccctcggacaccccgatcctcccacaataaaggcttctcaatccgcaaaaaaaaaaaaaaa

SEQ ID NO: 4 - DNA, 2883 bp, Homo sapiens
tcagccagtgtggcttcaggtcaagaggctgggcagggtcaaggtggcaacgaggggagaagccgggacacagttctccctgatttaaacccgggcagcctggagtgcagctcatactccatgcccagaattcctgcctcgccactgtcctgctgccctccagacatgctggggccctgcatgctgctgctgctgctgctgctgggcctgaggctacagctctccctgggcatcatcccagttgaggaggagaacccggacttctggaaccgcgaggcagccgaggccctgggtgccgccaagaagctgcagcctgcacagacagccgccaagaacctcatcatcttcctgggcgatgggatgggggtgtctacggtgacagctgccaggatcctaaaagggcagaagaaggacaaactggggcctgagatacccctggccatggaccgcttcccatatgtggctctgtccaagacatacaatgtagacaaacatgtgccagacagtggagccacagccacggcctacctgtgcggggtcaagggcaacttccagaccattggcttgagtgcagccgcccgctttaaccagtgcaacacgacacgcggcaacgaggtcatctccgtgatgaatcgggccaagaaagcagggaagtcagtgggagtggtaaccaccacacgagtgcagcacgcctcgccagccggcacctacgcccacacggtgaaccgcaactggtactcggacgccgacgtgcctgcctccgcccgccaggaggggtgccaggacatcgctacgcagctcatctccaacatggacattgacgtgatcctaggtggaggccgaaagtacatgtttcgcatgggaaccccagaccctgagtacccagatgactacagccaaggtgggaccaggctggacgggaagaatctggtgcaggaatggctggcgaagcgccagggtgcccggtatgtgtggaaccgcactgagctcatgcaggcttccctggacccgtctgtgacccatctcatgggtctctttgagcctggagacatgaaatacgagatccaccgagactccacactggacccctccctgatggagatgacagaggctgccctgcgcctgctgagcaggaacccccgcggcttcttcctcttcgtggagggtggtcgcatcgaccatggtcatcatgaaagcagggcttaccgggcactgactgagacgatcatgttcgacgacgccattgagagggcgggccagctcaccagcgaggaggacacgctgagcctcgtcactgccgaccactcccacgtcttctccttcggaggctaccccctgcgagggagctccatcttcgggctggcccctggcaaggcccgggacaggaaggcctacacggtcctcctatacggaaacggtccaggctatgtgctcaaggacggcgcccggccggatgttaccgagagcgagagcgggagccccgagtatcggcagcagtcagcagtgcccctggacgaagagacccacgcaggcgaggacgtggcggtgttcgcgcgcggcccgcaggcgcacctggttcacggcgtgcaggagcagaccttcatagcgcacgtcatggccttcgccgcctgcctggagccctacaccgcctgcgacctggcgccccccgccggcaccaccgacgccgcgcacccggggcggtccgtggtccccgcgttgcttcctctgctggccgggaccctgctgctgctggagacggccactgctccctgagtgtcccgtccctggggctcctgcttccccatcccggagttctcctgctccccacctcctgtcgtcctgcctggcctccagcccgagtcgtcatccccggagtccctatacagaggtcctgccatggaaccttcccctccccgtgcgctctggggactgagcccatgacaccaaacctgccccttggctgctctcggactccctaccccaaccccagggactgcaggttgtgccctgtggctgcctgcaccccaggaaaggagggggctcaggccatccagccaccacctacagcccagtgggtaccaggcaggctcccttcctggggaaaagaagcacccagaccccgcgccccgctgatctttgcttcagtccttgaatcacctgtgggacttgaggactcgggatcttcaggacgcctggagaagggtggtttcctgccaccctgctggccaaggaggctcctggggtggggatcaccagggggattttgacacagccttcggctgccccccactaagctaattccacacccctgtacccccccagggggccctctgcctcatggcaaaggcttgccccaaatctcaacttctcagacgttccatacccccacatgccaatttcagcacccaactgagatccgaggagctcctgggaagccctgggtgcaggacactggtcgagagccaaaggtccctccccagacatctggacactgggcatagatttctcaagaaggaagactcccctgcctccccagggcctctgctctcctgggagacaaagcaataataaaaggaagtgtttgtaatcccagcactttgggaggccgaggtgggcggatcacgaggtcaggagatggagaccatcctggctaacacggtgaaaccccttatctatgcgcctgtagtcccagctacccaggaggctgaagcaggataatcgcttgaacccgggcggcggagattgcagtgagccgaggtcatgccactgcactgcagcctgggcgacagagcgagattctgcctcaaaaataaacaaataaattttaaaaataaataaataataaaaggaagtgttagacaatgtaaaaaaaaaaaaaaaaaa

SEQ ID NO: 5 - DNA, 661 bp, Homo sapiens
agcatcccaaggcccgactccccgcaccactcagggtcctgtggacagctcacctagcggcaatggctgcaggaagaagcctatatcacaaaggaacagaagtattcattcctgcatgactcccagacctccttctgcttctcagactctattccgacatcctccaacatggaggaaacgcagcagaaatccaacttagagctgctccacatctccctgctgctcatcgagtcgcggctggagcccgtgcggttcctcaggagtaccttcaccaacaacctggtgtatgacacctcggacagcgatgactatcacctcctaaaggacctagaggaaggcatccaaatgctgatggggaggctggaagacggcagccacctgactgggcagaccctcaagcagacctacagcaagtttgacacaaactcgcacaaccatgacgcactgctcaagaactacgggctgctccactgcttcaggaaggacatggacaaggtcgagacattcctgcgcatggtgcagtgccgctctgtggagggcagctgtggcttctaggggcccgcgtggcatcctgtgacccctccccagtgcctctcctggccctgaaggtgccactccagtgcccaccagccttgtcttaataaaattaagttgtattgtt

SEQ ID NO: 6 - DNA, 10009 bp, Homo sapiens
cgtagctcataatccatttttataacaccttgctatctatatttacacctttaaagaacacgggaatttaagagggaagagtaactaggcttttgctaaacttgggctaataaaaccctctgtagagagatccttaatataggcatggggacaacaaggagtatcccaagggactcgccgctagggtgtcttttaagctattggagcaaattcaaatttggcttaaagaaaaagaaactcattttgtattgcaacaccatttgggttaaatacaagttagatgacgaatatatctggcctaaacatggttctatatactatagtgatattttacgattaggcttattttgtaaaagagaaggaaaatgggaagagatcccttatgtacaggcttttatggctctatactggatcacgttacttccaggcattagaatgccatgcataagggatccccacctagctgctccccatagaaagttcataagcctccccagagtctcttcagtcccccagtcctgagtgggggttctcgccaattccctaatgagattccaccccaatatcatcaggcacctttcccccttatccaactagccctagcctataccctctgctgcccaagaaaatgagcccaaccagtacaccaggagtggggctccatatcagcccctaaggtcaagcctgtgtccactgtggaaagtagttgatggaaatgagggaacactcaaagagtacatatgccactttccatgtctaattagaccttataaaaggaaagaattggccagttttcagataaaccagaaaagcttatacaagagtttgttacgttgactatgttcttcaaattgccacgatttacaaatattgtcatccgcttgctgtgctgtggggaaaaaaaagtagaggaaaaagtgtgtggttaagccagtcaattatgacaaggttaaagaagtaactcggggaaaagatgaaaatcccgctctgtttcagggtcttttagttgaagcactcaggaaatatactaatgcaggcccagacaccccagaagggcaagctctcctgggtatacattttctcattcaatcttctcctgacattaggaggaatctacaaaaagcagcaatgggaccttcaagtcctatgaaacgacgcttaaacatagcctttaaagtttacaacaacagggacagggcaaaagaggggagtaaaaagaaatagccaaaaagtacaattgttaacagtgactttaagcctccttgcccctcaggattactcatcttgagaaaatgttacaaaattagcatctgggatgcctagacaagacttgatgcctgacttgctgacccctgggccagaatcactgcgcctactatacgcaaaagggcccctggcaatgcaaatgtcctaactgctctggtgagagagaacaataacaacaaaaagcttccatcaatactagagctaaccttctcctactagccccagtgagctgcttagctcaagtaagtttactgtcccagaggacagctttccacagtggcagataagcagccgcctgaacatttttctttggtatttccaccactgagtgtgctctccagtggcgtggggactccagaatctccttttgagcaatgcagtttgcttcctcccctttttagttgatgctatgggattccctgtcctgccttttcctgttttccatacctatcggggcaaacaaaatttggccaggtagatgggtcccagttctgtaaataacttgaatccagttgtcttgtataggtcattttatttaatatgtttttgggtatatgtacatgtattgtgatgtgtgttacatctagcgtgctgtcaaactggcttatagataaaagaacactcatacattcaacaaataagactactgaaagcttattagtttgaagagaatcttgtatcttctaaaatttaactttaggatttttacctaggtaagtcactgatgttcataggctttaaaatggttaaaatggctttaaatggtgaccagctttgcatggtaccttggttctcggtgatctagataaagttaaaagtgaaataattaaatacacgtaaatgggatatgcttaatgtgtggtttaaaatcataaaatggtagaatggttctcagttatagaatgacaatgtctagtgtgaagttcatgacttcttccttcctaggtttccataaaatgtgctaaagaaatgtattctttattgagaaaaaattttttgtctaatccggaagttactaaatgggaggttcaaaacatgagtgaaccagtgagtagaaaagagagatgtaaagaatattatgaatagaaaatgtattttttgtttgttttgcaaggaaggatataaagaaagagtaattttatatgtggaggaatcctgtatagtaaattccctatcctagagtaaaataactttaagaaagaggtagtatagaacatgtcaggaaattcagctatgttgtagatggtctgtgtaagtcatctgcacagtgcatgagtgtggaggtgggcgggcactcattggcccttgaactccttttgagcagtatggaagccaagaactagaagccaggaaatggggttgtaaaactgatttgtctatggattttatgtgttgagctgctgtggtcttggcttgtagtaattacctatatgaaccttcccccctcccctttagaatttaggacaggttcaaaaggccctccaatataaaaataaaatactgtccttccccacaaaggaaaaaatagctccccggttcaaccaggagacttagtcttgctaaaaccttaaagacagggtaaagacagggataccccaagaatcaattacaatgaaatggaaggggccttatcaggtattgttaagtacccccactgctgttaaacttcagggaacacctacttgggcacacagatccaggactaaacctgtttcttatgagtcacaggcacaaaggaagggcactacaaccacaaccaatatcagtaaagctttggaagacctctgctacctatttaaaataatcaacactcagccagaagaggtaatgtaatgctgtagatgggaataggagcattgatcttgctcttcttcctgactgtagtacttcctttctatggctttaaccagccacctcctcctgggaaacatctcctgtgggcttgttgggtatagaagctactctaagacccaaccagataccatgatgccactgttaattctgtttgctcttctaattaacctaagctagtgtgtatgtggacagggagggtggacaaaattctacagtaaatatttcaaaaattatagcatcatagaatcatctttatggctgccagatttgtcatcaacacccccaggatagacagtttcatcttccgacctatctggaaaatctcaggaccatgtccccagacctcctaactaaccatagcaccccaaaatacccaaacccctattgtgaagtggaactcttccccacttagtggatcccccctggaccctgctgtccccctgccctgaccactattatcggaatctgggaagttgggcatctatatctccagtgcactcataactctaacatttgcatccactcttgcattaatgacacaaaagtggaagcttccctgcgatgctctggtccaactctagttgccaagtttccaagaccacggggaggtaaatgagattccatttgtgagtgaaaagaccatatatggtaccttctcccggatgggaacatacaaaggaaaaacaactgcctgatctgggaaggtgacagtactaccttcttctagaaaacaaagattgttcaaccaccaccatgagaacaggtggaaaatatctctatagacccaacctggcaatgaagtataaacatcgcaccccgcagggcttctcttggtgccctagttgggttcatttttgtttgtgactatgaatgggaagaagtcacaccctgtaaccactccaactccctaaggagtcacctcttctttaaggaatagctttcccttgtatctaaaaaacttggaactgacatgaatgaacgttggccactcttacccctccaggggtcacaatctataacgcctaggacccaagaatatcagaaataagtaagcaataaaactaattctggcaggaatcagggtggcaataggactagcagcaccctggggtggctttgcctaccatgagttaacgctaaagaacttggctcaaatcctagaatccttagccaccaacggagatcaggcattaaagagaattcaagagttccccagactctggaaaatgtagttgttgataacagactagcattggattatttactagctgaacaaggtggggtcttgtgcagttattaataaaacctgctgcacatatattaactctggacaggttgaggttaacattcaaaagatctatgagcaagctacctagttacatagatataaccagggcactgcccccaactatatctggtcaaccatcaaaagtgccttcccaagtctcacctgtttttcacctcttctaggacctttgacaactgtcttgttacaaatgtttggtccttgcttctttaacctcttagtaaagtttgtgtattctagattaccacagttccagagacaatgctggcacaaggcttccagcccatcctgtccactgacacggagaatgaaatcgtcctgcctctgggctccttagatcaggtatccagagatttttactcctccagtgccaggcagggcctacgtccataaactcagcaggaagtagttacggaaaacagatctccgcccttctgcagcccccttaagattaaggaggagtatctaatctctgaagggggaatgaggtaggaggtgggactcaactctggaagtggggctcaggcactcagaccaaactgagcactagctaaaataggtccagggcagatgctagtttccataggacacaccgacctgtgtcaagtcagttcaccatggctctggcagcacccagaagttaccaccctcaccctggaaatgtctgcataaactgccccttcatttgcatataattaaaagtggatacaaataccactgcagaactgcctctgagctgctactgtgggcgcacagcctgtagggcagccctgctttgcaaggagcagcgcctctgctgctgctgtgcacagccggccgcttcaataaaagttgctaacaccactggcttgcccttgagttccttcctgggcaaagctaagaaccctcccgggctatgcttcaatcttagggctcgcctgtcctgcatcactgggatcatctcccagtaaactagccacacttacatccatgtgtcagggacatttctggagaaagcagcccaggacactgttgaataaaacacacaatagtctctgtggtcttctccaccccaccccacaccaggcaccctcagcttgattctcctttttaattgcctgtaagcagggaagcacaatgttttcacattctttgtaaggcctttgttctactaaaatctaacctcagagcacaattttaaactagatgaaagagttgctgcgcctgaagcactgcaaacacctcctcaccacacatgtgcactcaccctggacaccctcactcaccctgacaccctcactcctcaccctggacaccctcactcaccccagacaccgtcactcctcaccctggacacctcactctgcaccctggacaccctcactcaccctggacacgttcactcaccctgacaccctcactcaccctggacaccctcactcaccctggataccctcactcctcaccctggacaccctcactcaccctggataccctcactcctcaccctggacactctcactcaccctgacaccctcaatcctcaccctggactccctcactcctcaccctggactccctcactcctcaccctggacaccctcactcctcatcctggacaccctcactcaacctggacaccctcactcctcaccctgacaccctcactcctcaccctggacaccctcactcctcaccctgacaccctcactcctcaccctggcaccctcagtcaccctgacaccctcactcctcaccctgacaccctcaagtcttcacctccctggctgcagcctgggacacgctttccctaacttctgaaggctcagtcctcctcaagccaatctcatctcaaattgcacctcctcagagaggtcttccataaccgcccttataaagcaggattctttcaccaataccccttcccacatggcactgtctcacagcactcctctaaaagtctgtttacttccttgacaatctgtcttccttataaggggaggttctgtaaaagccaagactctctctgtctagttgactgttgcataccagggcttagaccaaggccctgacatgcagtaggtgcttaatatgttttgaggcaaggtcttgctctgttgcacatgctggagtgcagtggcacaatcgtaattcattgcagccttgaactcctgagctcaagtgatcctcctgcctcagcctcctgagtagctgggactacaggcatgcaccaccaagcttggctaatttaaaaaaaaaattatatagatagggacttgctatgttgcctaggctgatcttgaactcctaacctcaagcaatcctcccacctcggccttccaaagtgctgggataataggcatggagccgccacacccagccaatgtgccgaagaaagaaagaaaaacatgctcatcctttgagtcaggttcaaattttttctcctctttaacccccagtcactccagttataagtgatttttaactcttctcacactttaatgcatctggcaagaagatccacgtggtgttaggaacaatacaggaccttaaggatgggggaatcagcaggtgtcagcgtgccctgtatgctcagggcagctgtttccactggacattctccctttgcctctctgggcagcaactcctaggccagccgacctgctgtgtcgagtaaccaggatttctcaatcttggcatggttgccattttggaccagatcgttctttgttgtgggggctgccctgtacggcaaagaatgccgagcagcacttccagtctccacccacaggacgccagtagcaccctctaagttgtgagaactcaaaatgtccccagaggatgccagatgtcccctggggtggggacacaatcaccccaggttgagatccatggagccaggtctgtttgccaccaaggggtaaagctccattcccaccttaggagggctaggaggcagcatcgtggggccacagaaggcctgggtttgcagtcagaggacaggatgcacattccttcaagatacagacccagattgttgggcatctagttcttgggttttctgttgttgctgttccgttttgtctgtcttccctcctttgtttactagcagcctggaatttgccactttttctaaacgaagatttatggaacacttaccacacggctgacgctgcgcgaggctaaggttctaatacaccgcagctcacttaactctcgcaataccataaacgcacactgtttcatcttgaccctttcttgggaaggtgacagagaggtaggagggcaaacatcttgtgtgccccgtcccaagggtattactggtggaataatatccgccccccaccccagtttctaatttgctgtaggctgtgacgctgtggggcaagactaggagtcctgttgaaattaggaataagtgtgctgtgagggaagggctgccttattttagagcacagattttctgaatatctattttgacaggttcgatcctctccccttcctgccttccttctgtcgattttcaatgtcttgatggtgtcccacctgagtggcctttagagatgtgagttgtgaggcactggggaggcaggcacacgtcctccagcccaagactgcctaatttaacagggatttctgcattctggaacaagcctccattttccccaagcaggattactccagagggcaaaacacagcccaatagtatcacatttcctttctgctttagcaaaaataaccactgtctcattcatgggaaaaggccgccaaacaaatttgttactggaaccatttgtaacaacttctagtttgcactgccttggagcaagcacactttgtagaggagggatttgcagttacttgggcaacaaggtaaccactgatcattacaggaagcttcagaaaccgtgggaccagtgtagaagaatggactatctgtccaaactaagaataaaaagaatgacacttgtattttgtatgtctttttcactttgcctttctagtaattcatttttcttgatatttacaccttgtggccctgtgatagactggaaatctcaaaaacacacgttcagcaccaagattttcagcagcaccgcctcagaatgagacccctagaaaaaactgcgtgttttccacttgcccaacacgaggagtttttggaacacgacctgcttgaggtggagattttctagatgggcaaagagaaggaaacacttaacctaggaagagtatttaggaagaagaaagaacacagcctttctgcacaggaaaccgccgagcagaggggcatctggcctctgcagtggcctccaaatagagtccaatggctggggccagcgtggctgcttaaaggggactcaagggatataataaaatgcagattctcaggtcctagtgcagacaggctcacccaataagtctggactgcatatgggaatctctatttctaggcccttctgcaaggtattcctgctctttccaggaaccatcggcagctggtttggggaaagaagcaacgactccaagtgtgacctgtgagctggcagcagccaccctcagctctgctctcggtcactgaatccgattctgcattttaacaggaccccaggtgttgcacccacacaaagctgaagcagattggtctgggggcaaaaaattagagctatggagattctctcaaatgaaatagatgatatcattgactgttagagcttctagaaggaatctgaggtcacttgttcaaattccctgatttacagatgaggaaacagaggctcagacagctcaaatgacttctctccaatacccaacattcgacaagtagcagctctgggactagtacccaaagcacctagctctccaatcactgcgcaagccacacaattctgtctgcttgtcagtggcttttctgattcaaaaaaagcttaggaatttccccaggaggcagcacgatgtagtgggaagggctctggatgtctctccaaggcttctggaattcatgcccacctccaccaagaagccactttcctgccagctacaggtgctcacctgaaaagcaagccagaccatattaaccctggcattgctggtacctggaagactttctgattcaatgctttccacctcctcctacccctcaccacccccgtggcatgaaatcctgggggctgctttagaaattgttttctttggctgctggtgggggtgctgctggtgggggtttgcacagctggcacactgcaccagtctggtgggggtttgcacagctggcacactgcaccagtctcctgcctgctgccaacaaggccatttcccaagcactggctttggagaagttggggctctgaagtgggaacacaaggctgccttttgcaggccaggtgtaaattctccccctgccactttcagcctagcgtgaaacagatggagtgtgcattcccacttccctttatggtaccctggaatgatggagctgcccagggcatcgccacgttactctctagacagtctctttgtcttcctgcaatggcagcgccgaggttgtatatttctaggtgcaggtatatgattgccatataataaaaatctgaaaacatccca

SEQ ID NO: 7 - DNA, 2046 bp, Homo sapiens
agtgcagaaggaggaaggacagcacagctgacagccgtgctcaggaagattctggatcctaggctcatctccacagaggagaacacgcagggagcagagaccatggggcccctctcagcccctccctgcacacagcatataacctggaaagggctcctgctcacagcatcacttttaaacttctggaacccgcccaccacagcccaagtcacgattgaagcccagccaccaaaagtttccgaggggaaggatgttcttctacttgtccacaatttgccccagaatcttactggctacatctggtacaaaggacaaatcagggacctctaccattatgttacatcatatatagtagacggtcaaataattaaatatgggcctgcatacagtggacgagaaacagtatattccaatgcatccctgctgatccagaatgtcacccaggaagacacaggatcctacactttacacatcataaagcgaggtgatgggactggaggagtaactggacgtttcaccttcaccttatacctggagactcccaaaccctccatctccagcagcaatttcaaccccagggaggccacggaggctgtgattttaacctgtgatcctgagactccagatgcaagctacctgtggtggatgaatggtcagagcctccctatgactcacagcttgcagctgtctgaaaccaacaggaccctctacctatttggtgtcacaaactatactgcaggaccctatgaatgtgaaatacggaacccagtgagtgccagccgcagtgacccagtcaccctgaatctcctcccgaagctgcccaagccctacatcaccatcaataacttaaaccccagggagaataaggatgtctcaaccttcacctgtgaacctaagagtgagaactacacctacatttggtggctaaatggtcagagcctcccggtcagtcccagggtaaagcgacgcattgaaaacaggatcctcattctacccagtgtcacgagaaatgaaacaggaccctatcaatgtgaaatacgggaccgatatggtggcatccgcagtgacccagtcaccctgaatgtcctctatggtccagacctccccagaatttacccttcattcacctattaccattcaggacaaaacctctacttgtcctgctttgcggactctaacccaccggcacagtattcttggacaattaatgggaagtttcagctatcaggacaaaagctttctatcccccagattactacaaagcatagcgggctctatgcttgctctgttcgtaactcagccactggcaaggaaagctccaaatccgtgacagtcagagtctctgactggacattaccctgaattctactagttcctccaattccatcttctcccatggaacctcaaagagcaagacccactctgttccagaagccctataagtcagagttggacaactcaatgtaaatttcatgggaaaatccttgtacctgatgtctgagccactcagaactcaccaaaatgttcaacaccataacaacagctgctcaaactgtaaacaaggaaaacaagttgatgacttcacactgtggacagcttttcccaagatgtcagaataagactccccatcatgatgaggctctcacccctcttagctgtccttgcttgtgcctgcctctttcacttggcaggataatgcagtcattagaatttcacatgtagtataggagcttctgagggtaacaacagagtgtcagatatgtcatctcaacctcagacttttacataacatctcaggaggaaatgtggctctctccatcttgcatacagggctcccaatagaaatgaacacagagatattgcctgtgtgtttgcagagaagatggtttctataaagagtaggaaagctgaaattatagtagactcccctttaaatgcacattgtgtggatggctctcaccatttcctaagagatacattgtaaaacgtgacagtaagactgattctagcagaataaaacatgtactacatttgctaaaaaaaaaa

SEQ ID NO: 8 - DNA, 11025 bp, Homo sapiens
gagcatcttttggggggagggaattcagcggatcagtcttaagaggagcttttttttggagcgagaaatcatataaaataaaatgaaataaaacaaggaggaaggcaaccagctgttaggggaaaaataaggcagataaaggagcggggagagaaattaattgccaaccaggaggagttgggctgtatttttcaaaggtggggagagtggagcacacaccttgaggaggaaagcgagaaagaaaagaaaaaagcaagtggaaaggggggctcgcccaagaagggtgaagaagcgaagaaagtcgaggcgccgaggctcccaaagctggcagctccgggtggcggtgcaggggcgaagggggggcggggggaaccgtcggacatgcggctctggagttgggtgctgcacctggggctgctgagcgccgcgctgggctgcgggctggccgagcgtccccgccgggcccggagagacccgcgggccggccgacccccgcgccccgccgccggcccggccacctgcgccacccgggcggcccgcggccgccgcgcctcgccgccgccgccgccgccgccgggcggtgcctgggaagccgtgcgcgtcccccggcggcggcagcagcgggaggcgaggggcgccaccgaggagccgagcccgccgagccgggcgctctatttcagcgggcgaggcgagcagctgcgcctccgggccgacctcgagctgccccgggacgcgttcacgctgcaagtgtggctgcgagcggaggggggccagaggtctccggcagtgatcacagggctgtatgacaaatgttcttatatctcacgtgaccgaggatgggtcgtgggcattcacaccatcagtgaccaagacaacaaagacccacgctactttttctccttgaagacagaccgagcccggcaagtgaccaccatcaatgcccaccgcagctacctcccaggccagtgggtatacctagctgccacctatgatgggcagttcatgaagctctatgtgaatggtgcccaggtggccacctctggggaacaagtgggtggcatattcagcccactgacccagaagtgcaaagtgctcatgttagggggcagtgccctgaatcacaactaccggggctacatcgagcacttcagtctgtggaaggtggccaggactcagcgggagatactgtctgacatggaaacccatggcgcccacactgctctacctcagctcctcctccaggagaactgggacaatgtgaagcatgcctggtcccccatgaaggatggcagcagccccaaagtggaattcagcaatgcccacggctttctgctggacacgagtctggagcctcctctgtgcggacagacattgtgtgacaacacagaggtcattgccagctacaatcagctctcaagtttccgccagcccaaggtggtgcgctaccgcgtggtcaacctctatgaagatgatcataagaacccgacggtgacgcgcgagcaggtggacttccagcaccatcagctggctgaggccttcaagcaatacaacatctcctgggagctggacgtgctggaggtgagcaactcctcccttcgccgccgcctcatcctggccaactgtgacatcagcaagattggggatgagaactgtgaccccgagtgcaaccacacgctgacgggccacgacggcggggattgccgccacctgcgccaccctgccttcgtgaagaagcagcacaacggggtgtgtgacatggactgcaactatgaacggttcaactttgatggtggagagtgctgtgaccctgaaatcaccaatgtcactcagacttgctttgaccccgactctccacacagagcctacttggatgttaatgagctgaagaacattcttaaattggatggatcaacacatctcaatattttctttgcaaaatcctcagaggaggagttggcaggagtagcaacttggccatgggacaaggaggccctgatgcacttaggtggcattgtcttgaacccatctttctatggcatgcctgggcacacccacaccatgatccatgagattggtcacagcctgggcctctatcacgtcttccgaggcatctcagaaatccagtcctgcagtgacccctgcatggagacagagccctccttcgagactggagacctctgcaatgataccaacccagcccctaaacacaagtcctgtggtgacccagggccaggaaatgacacctgtggctttcatagcttcttcaacactccttacaacaacttcatgagctatgcagatgacgactgtacggactccttcacgcccaatcaagtcgccagaatgcactgttacctggacctggtctaccagggctggcagccctccaggaaaccagcgcctgttgccctcgccccccaagttctgggccacacaacggactctgtgacactggagtggttcccacctatagatggccatttctttgaaagagaattgggatcagcatgtcatctttgcctggaagggagaatcctggtgcagtatgcttccaacgcttcctccccaatgccctgcagcccatcaggacactggagccctcgtgaagcagaaggtcatcctgatgttgaacagccctgtaagtccagtgtccgcacctggagcccaaattcagctgtcaacccacacacggttcctccagcctgccctgagcctcaaggctgctacctcgagctggagttcctctaccccttggtccctgagtctctgaccatttgggtgacctttgtctccactgactgggactctagtggagctgtcaatgacatcaaactgttggctgtcagtgggaagaacatctccctgggtcctcagaatgtcttctgtgatgtcccactgaccatcagactctgggacgtgggcgaggaggtgtatggcatccaaatctacacgctggatgagcacctggagatcgatgctgccatgttgacctccactgcagacaccccactctgtctacagtgtaagcccctgaagtataaggtggtccgggaccctcctctccagatggatgtggcctccatcctacatctcaataggaaattcgtagacatggatctaaatcttggcagtgtgtaccagtattgggtcataactatttcaggaactgaagagagtgagccatcacctgctgtcacatacatccatggaagtgggtactgtggcgatggcattatacaaaaagaccaaggtgaacaatgcgacgacatgaataagatcaatggtgatggctgctcccttttctgccgacaagaagtctccttcaattgtattgatgaacccagccggtgctatttccatgatggtgatggggtatgtgaggagtttgaacaaaaaaccagcattaaggactgtggtgtctacacgccccagggattcctggatcagtgggcatccaatgcttcagtatctcatcaagaccagcaatgcccaggctgggtcatcatcggacagccagcagcatcccaggtgtgtcgaaccaaggtgatagatctcagtgaaggcatttcccagcatgcctggtacccttgcaccatcagctacccatattcccagctggctcagaccactttttggctccgggcgtatttttctcaaccaatggttgccgcagctgtcattgtccacctggtgacggatgggacatattatggggaccaaaagcaggagaccatcagcgtgcagctgcttgataccaaagatcagagccacgatctaggcctccatgtcctgagctgcaggaacaatcccctgattatccctgtggtccatgacctcagccagcccttctaccacagccaggcggtacgtgtgagcttcagttcgcccctggtcgccatctcgggggtggccctccgttccttcgacaactttgaccccgtcaccctgagcagctgccagagaggggagacctacagccctgccgagcagagctgcgtgcacttcgcatgtgagaaaactgactgtccagagctggctgtggagaatgcttctctcaattgctccagcagcgaccgctaccacggtgcccagtgtactgtgagctgccggacaggctacgtgctccagatacggcgggatgatgagctgatcaagagccagacgggacccagcgtcacagtgacctgtacagagggcaagtggaataagcaggtggcctgtgagccagtcgactgcagcatcccagatcaccatcaagtctatgctgcctccttctcctgccctgagggcaccacctttggcagtcaatgttccttccagtgccgtcaccctgcacaattgaaaggcaacaacagcctcctgacctgcatggaggatgggctgtggtccttcccagaggccctgtgtgagctcatgtgcctcgctccaccccctgtgcccaatgcagacctccagaccgcccggtgccgagagaataagcacaaggtgggctccttctgcaaatacaaatgcaagcctggataccatgtgcctggatcctctcggaagtcaaagaaacgggccttcaagactcagtgtacccaggatggcagctggcaggagggagcttgtgttcctgtgacctgtgacccacctccaccaaaattccatgggctctaccagtgtactaatggcttccagttcaacagtgagtgtaggatcaagtgtgaagacagtgatgcctcccagggacttgggagcaatgtcattcattgccggaaagatggcacctggaacggctccttccatgtctgccaggagatgcaaggccagtgctcggttccaaacgagctcaacagcaacctcaaactgcagtgccctgatggctatgccatagggtcggagtgtgccacctcgtgcctggaccacaacagcgagtccatcatcctgccaatgaacgtgaccgtgcgtgacatcccccactggctgaaccccacacgggtagagagagttgtctgcactgctggtctcaagtggtatcctcaccctgctctgattcactgtgtcaaaggctgtgagcccttcatgggagacaattattgtgatgccatcaacaaccgagccttttgcaactatgacggtggggattgctgcacctccacagtgaagaccaaaaaggtcaccccattccctatgtcctgtgatctacaaggtgactgtgcttgtcgggacccccaggcccaagaacacagccggaaagacctccggggatacagccatggctaaggaaggacaagaagttgtcaaagaattcccaacgccaggacccacatccctttggtattgatttcacagtcagctgctcaacggaatggcctctccacaccagggatccttagcacccaaccggtctgcctttaattttacccaggaaggactcacattggggcgaatgaaccaagtttcgccatgctggatgatgaaatggattcccatcccaaagtctgagatggattgcatatacagtgtgcagtcccagagcctcctaaaattctagccatttgtcacacaaccacagcaagaaacgtgttctatatctagagtgtgcccatctgtgtttagtacacatgcatgcatacacacccatacaaacatctgtgtgagggcagttctggagatgagcagagagagaccggaataaactcaatcttttctttcccaagctcctagccaacactatccttgggagaaagaaatttgcagaaactgctaagaccaagtgtggagatgtcaagctagttcacactctgaggctcagaatatgtaggacatgcacaattgtgcagtcctttgggattggaagtgaaacagtctgtgatcccctaccttctagggaactaggacctaggaagaggtaaagattatcaggtatgcaaagcgccccaattcttctgctgccatgggggattttaccccaactccagggttcgaggccaatctgagaatggcttaggattgcaatgtcaaggtattatatcagccccttgcttgaggcttgaggtcataatatccctctaggacttacctgttcccccagatcttgccttgggaccacatttgctgctacttttcctgctgctctatcctatacattgaataatccaagatggtagaactaggttaggaaaaattccacacaaccaaacagtctgccttaaaagtgacccacatttttccatagctcctcactttttagcccttctgcaagagaaaaaccctcatgggtccacatggtgagaagttaagtttcctgtaagtgggcctctcaccctggaaaggagttgagggacatcagatgctggaaccctcactgaaagtccagaatgtctaagccagtgttagattttgtaaacaagtggaacagtgttaaatttctatgatgttggagccatccagagactactggaattgtcgagacttttggattattatccttatccttatcctaatcttcctagcccttcaggctagagtaggcttcgatcctgagaaccttgctgttgctctgaggagatataattctgggagaaagaatcttttataagaacagtacagattgttctcaagagggccatcagaaggaagccaaagagttcacagcctcagcaccaacaactcaacatggtcatcatgttttctatatggtttttccagctagcagtactcccttccatacctgtgactgggcagtgcttttctctctcccatgtctagcctccaaaagttaagtgaaaattagtcaactgcacgtggaagcccccaccactttggggatctctttatttcttttcagccagggacctgtccactccctttgaattaatatgggaagaaattaatacaggatgaactggagagaagggttgagtgtggcatactttctgaaacctggagctgggaattgcggagaagggaaggtctagactagttacatcacatagggattactgtaaatcaagtcatctcaagtctagtgaagacagccaacagaaacaaaacctagcatagggatagaaaataccatgcacgtgtgcagccccacctaattcctgcatccaaggcaggtgttgttaatctatcatagcacttaaaaaaaaaaaaaaaaagagaccaaaaataactttaggaaccaccatattatatcactcccaatagcactgacctggtgatcaaaaacacttgagaagacatctattggccatctctggccaattacactaagaaacatatcaaggtgcttttggcacaggtgcccacaaatacggatgcagtgctgagatagtttatgagacttgtaccatttcacaaactctgaaattgggttccatattggcaaggctgccacagttgttaagaataatcctctatgtttcttcctcacaaaaccatatctcatttatatccagaccattacttcactataattacaaggacaaattattagcaagaaataagaatagtattagaagaattgatcctattttgaacccctctccagtatcttcacactcttgtcaactctccaggcctctctcttgccctgagttatcagcctgtgtggtgttaactaccttagaaggtacaagctaagaaatgtaacagtatcaaccctcccagttgcttaattatacccataggtaatacaaaaagctctgaagacccaaagatgacattactaatgatgtgatttcaggagccacagaagaaccttaccagcttccctcaaatcagtccttatcctctttctatcttcactcccatcatcatctattttcacactatccagctaagcaaagattcctggaggctgacttgtatcttcagactcacagagtgaattcagctcttctgaatcaagacccacccagtctctttcattcagacctgttgctaacaaatttatatttgccaaggatattaggcaaaagaggctacttgattggtggccaacctcgtgcccacatggaaggtatctttaatagggtcttttcaaaccttagtggaggagggtcagctcaatttgggcaatgcatttgttcccagtttcattttcttcctgggaattaactcgtcatttcattccttcagtcatcttctgtgtaggtgaccggagcactgagaggcagctctgatgcactattgtgtgtcagcagctcaaaggccctaaaacactgaaggttctgcatctgaagtattagattgttagcagcaaaatatgaaagatgaggtggacagtcctctaagccctatttagggaagcttttccaagccacaatcttaactacctacccaaaggatttgcattacccccagattctgtgccaacaaccttttaaggaaatacagtccttgggaaatgagttttgatggtgaattggggtgttaaggaagggaaagattgtcatagatggtagggctttgaaaatgcagggtatcagctgccactcctggcttcaacacattgagtcactgcctagacggttctcttggtcttattcccatcctggccaatgcttaaatactatttgttgaaaataattctttgagacagatttcagctacctcccttccaggttcgatttaacttggttgtaattgtcaatttgttgttataggtcttacctgtgtgaaagaaagaaaaagaaagaaagaaagaaagagaaaggaaattataaggtcaagttaacagttttgaggttttgtgtttttttctggaactacttcaagtgagaaaataaaaaaaaatggtgacaaagctgtacagatagagataatagaagacaaagagattaaaaggaaataaaaatgcatgattaaaaactaagaataaaaaacctatttttatgtttcctaaaggaaattgtttattctacagcctcagtaggtagacacaaacataaagatttccctagaagacatagagtgggatttgataacactgtctgttattttctgtacattgtggtaggtccaggaaatatgacattttcccccttgatgtgttattgttgttgttgggtggggtgggcattttgtttatttgtttggtggcaatcagtggtagtagggagtgggagggcttatattggtttttccagctattaaggggacatattgtgtcgttgtgcttttcacgttataaaatgtttatatttaccagtacagcactgggctttataaagactgcactcagaaccacactgcacagtccagttttttaaaaagctgctacatgacagacaggtaatcccactgagtgagttttgagaaacaaatcaaacgaagtaaacaagaaacataaaaaccaaatagcaaatgaataaaagcctgttcttgtaacttattcaacttttgccaaattcctaccaatcacttgctttttaaaagaaatgtataatagccaaaagagaaattatgtccctgttgtacagaagttagaatttttgactccaggcagcagtttgctcagtgatcttgaacaagttatccaattgcctctacatttgcatcagtttctctagctgcaaaatggggataatactatatacctacctcacagtgggagggcaggagattttgaggccctgaggttttaggtgggctgtgagggccaacgcttgacacaaagtccatgggttattattcaagaatgcacaggcccatcggccttttagaaagacaagacagggagtgcttgtttgatatttcaaggaataaagccggagctcctgaattgtagtccaccttaaaagagagacctgtattggagaatattttatttttttggcaaatttgatcttaccctttaccagttctataatttggttaaaagctgattatgtcctacaatgtcaaagtcagctaactgtcgtctacttaagacttctggtcatttccaacttatagaggaagggagtctctaaaatctcttcttcagaaggcacctcacttctcagacttaaaattccacatcaagtgttccattaaaagaagataaggcattctgagtgcaaacaaatgggggcttcttaaactacacaccagcagtcagtgaggaaaactttgaacaattattgagttgctttcttgggtctctataatcaataacctgtctgcagatatctatctatataaagatattatatataaatataaatttacatatatatgcacatgtatatatagttgtacatatatgtgtgtatatatatacttaaatgtaatatttacaaaataaaactgtgatctcgtctagagaaaatgtattcatattacaaactgctcttccatatttatgtaccatattatacctttttattattgttataattattatgggtatttctaattaatatgatgttgaaacctgtttggcaccttctggaagctaccaaaaaaatgacactccattgaagtgcttaaaagctgttctcataagaattctactggcctattgtaaaaaagaaaaaaaaaaagaaaaagaagaaagacacaaagaaaataatctaaacaccaaaaactaaacacaattccaatcctttttctgtacctcacgcgcataaatttgctgctcctatttttttttctgtttatgtgtttttatggatctaagttaaatcttttggcaatatataaaaatgtaaatagtaaactttatttattaagaatgtcatcttttttaatttatatttacacaattgttcatctaatttattttttctatacagttttaaatactcagacatattttgctgttcatgatatttttatcctgttctcatggatttgttttcccatactgttttctctgatctcaattacaggttggatctcacaaataataatgtcagagacagaaatattttgccactgttgattactatactttaaagttctatattatgaaaatatataatagcttgtacgcttcaaaaaaaaaaaaaaaaaaaaaaaaaaaaaaaaaaaaaaaaaaaaaaaaaaaaaaaa

SEQ ID NO: 9 - DNA, 794 bp, Homo sapiens
gctgcattacagacacagacctgcaaacatctatggttgtgacagagtttctttctgacacctgagtctttctcctgctgcacggaaagcttgctgggaggggcttggaatctggcatgaagccaaagggcatctctgagttgcagcatttaaatgatcccactcagagattcacacagaagactggacacaattccgaagagctgcccagaaggagagaacaatgtcatcactacccgtaccatacacactgcctgtttccttgcctgttggttcgtgcgtgataatcacagggacaccgatcctcacttttgtcaaggacccacagctggaggtgaatttctacactgggatggatgaggactcagatattgctttccaattccgactgcactttggtcatcctgcaatcatgaacagttgtgtgtttggcatatggagatatgaggagaaatgctactatttaccctttgaagatggcaaaccatttgagctgtgcatctatgtgcgtcacaaggaatacaaggtaatggtaaatggccaacgcatttacaactttgcccatcgattcccgccagcatctgtgaagatgctgcaagtcttcagagatatctccctgaccagagtgcttatcagcgattgagggagatgatcagactcctcattgttgaggaatccctctttctacctgaccatgggattcccagagcctactaacagaataatccctcctcaccccttcccctacacttgatcattaaaacagcaccaaacttcaaaaaaaaaaaaaaaaa

SEQ ID NO: 10 - DNA, 6299 bp, Homo sapiens
gtgacgtcacgcgtcgacgctggggcgtacctttcgggctcctgactcctgccgcttctcttccccttccgtgggtcagggccggtccggtccggaacctgcagcccctttcccagtgttctagttcgcccgtgacccggaataatgagcaaggagggtgtggtgggttgaaagccatcctactttactcccgagttagagcatggattcagttttagtcttaagggggaagtgagattggagatttttatttttaattttgggcagaagcaggttgactctagggatctccagagcgagaggatttaacttcatgttgctcccgtgtttgaaggaggacaataaaagtcccaccgggcaaaattttcgtaacctctgcggtagaaaacgtcaggtatcttttaaatcgcgatagttttcgctgtgtcaggctttcttcggtggagctccgagggtagctaggttctaggtttgaaacagatgcagaatccaaaggcagcgcaaaaaacagccaccgattttgctatgtctctgagctgcgagataatcagacagctaaatggagtctgagcagctgttccatagaggctactatagaaacagctacaacagtataacaagtgcaagtagtgatgaggaacttttagatggagcaggtgttattatggactttcaaacatctgaagatgacaatttattagatggtgacactgcagttggaactcattatacaatgacaaatggaggcagcattaacagttctacacatttactggatcttttggatgaaccaattccaggtgttggtacatatgatgatttccatactattgattgggtgcgagaaaaatgtaaagacagagaaaggcatagacggatcaacagcaaaaagaaagaatcagcatgggaaatgacaaaaagtttgtatgatgcgtggtcaggatggctagtagtaacactaacaggattggcatcaggggcactggccggattaatagacattgctgccgattggatgactgacctaaaggagggcatttgccttagtgcgttgtggtacaaccacgaacagtgctgttggggatctaatgaaacaacatttgaagagagggataaatgtccacagtggaaaacatgggcagaattaatcataggtcaagcagagggtcctggttcttatatcatgaactacataatgtacatcttctgggccttgagttttgcctttcttgcagtttccctggtaaaggtatttgctccatatgcctgtggctctggaattccagagattaaaactattttaagtggattcatcatcagaggttacttgggaaaatggactttaatgattaaaaccatcacattagtcctggctgtggcatcaggtttgagtttaggaaaagaaggtcccctggtacatgttgcctgttgctgcggaaatatcttttcctacctctttccaaagtatagcacaaacgaagctaaaaaaagggaggtgctatcagctgcctcagctgcaggggtttctgtagcttttggtgcaccaattggaggagttctttttagcctggaagaggttagctattattttcctctcaaaactttatggagatcattttttgctgctttagtggctgcatttgttttgaggtccatcaatccatttggtaacagccgtctggtccttttttatgtggagtatcatacaccatggtacctttttgaactgtttccttttattcttctaggggtatttggagggctttggggagcctttttcattagggcaaatattgcctggtgtcgtcgacgcaagtccacgaaatttggaaagtatcccgttctggaagtcattattgttgcagccattactgctgtgatagccttccctaatccatacactaggctaaacaccagtgaactgatcaaagagctttttacagactgtggtcccctggaatcctcttctctttgtgactacagaaatgacatgaatgccagtaaaattgtcgatgacattcctgatcgtccagcaggcattggagtatattcagctatatggcagttatgcctggcactcatatttaaaatcataatgacagtattcacttttggcatcaaggttccatcaggcttgttcatccccagcatggccattggagcgatcgcaggaaggattgtggggattgcggtggagcagcttgcctactatcaccacgactggtttatctttaaggagtggtgtgaggtcggggctgattgcattacacctggcctttatgccatggttggtgctgctgcatgcttaggtggtgtgacaagaatgactgtctccctggtggttattgtttttgagcttactggaggcttggaatatattgttccccttatggctgcagtcatgaccagtaaatgggttggagatgcctttggcagggaaggcatttatgaagcacacatccgattaaatggataccctttcttggatgcaaaagaagaattcactcataccaccctggctgctgacgttatgagacctcgaaggaatgatcctcccttagctgtcctgacacaggacaatatgacagtggatgatatagaaaacatgattaatgaaaccagctacaatggatttcctgtcataatgtcaaaagaatctcagagattagtgggatttgccctcagaagagacctgacaattgcaatagaaagtgccaggaaaaaacaagaaggtatcgttggcagttctcgggtgtgttttgcacagcacaccccatctcttccagcagaaagtcctcggccattgaagcttcgaagcattcttgacatgagcccttttacagtgacagaccacaccccaatggagatcgtggtggatattttccgaaagctgggactgaggcagtgccttgtaactcacaatgggattgtcttggggatcatcacaaagaagaacatattagagcatctcgagcaactaaagcagcacgtcgaacccttggcgcctccttggcattataacaaaaaaagatatcctccggcatatggcccagacggcaaaccaagaccccgcttcaataatgttcaactgaatctcacagatgaggagagagaagaaacggaagaggaagtttatttgttgaatagcacaactctttaacctgagggagtcatctacttttttttcctcctttacaaaaaaagaaaggaaatataaaagccgggtttttgcaacatggtttgcaaataatgctggtggaatggaggagttgtttggggagggaaaggagagagaaggaaaggagtgaggtatttcccgtctaacagaaagcagcgtatcaactcctattgttctgcactggatgcattcagctgaggatgtgcctgatagtgcaggcttgcgcctcaacagagatgacagcagagtcctcgagcacctggcctgttgctccaacattgcaaagacacattatcagtccctatttctagagggattactttgaattgagccatctataaaactgcaaggtcttgcccttttttttaatcaaaactgttctgtttaattcatgaattgtatagttaagcattacctttctacattccagaagagcctttatttctctctctctctctctctctctctctctctctactgagctgtaacaaagcctctttaaatcggtgtatccttttgaagcagtcctttctcatattgagatgtactgtgattttactgaggtttcatcacaagaagggagtgtttcttgtgccattaaccatgtagtttgtaccatcactaaatgcttggaacagtacacatgcaccacaacaaaggctcatcaaacaggtaaagtctcgaaggaagcgagaacgaaatctctcattgtgtgccgtgtggctcaaaaccgaaaacaatgaagcttggttttaaaggataaagttttcttttttgttttcctctcagactttatggataatgtgaccgggtcttatgcaaattttctatttctaaaactactactatgatatacaagtgctgttgagcataattaaataaaatgctgctgctttgacagtaaagagaaggaagtattctgattagctgtatctggtattaattgcatgttaaaacactggaatttttaaaattgaaattagatcagtcattcttttcttttctcaagatatctcatggctgacactgaagaagaaatgtaattcataacttgcactaaatgtatattttttttcttaaaaatttaccattcttatttatatttttatggattaaaatttataaaatacagatcagttaatattgcacttaagtaattttacctttttaatgtgatttttatagaataattcagacttacaaatacagagatatgaacaaagtttacagtgggaacaaaggtttaaaaaaaggttgtggttctctctctgtgatccagtgtgcacataaacctttctctgatctttcactgccatcctctggattatgtcttctgacctgtccattttgacccattaactggaaagttgaaaaactacattaactggaaagttgaaaaactacattactttggagaataaaaccgaaagttcgtgtataccttcttaaaaaaaaaatcaaaccaaaaatgtgaaaacaatagaattgcaaagatagcagttaaaattttaatctgaaaataacctttgaatctcgggctaggttacgtccatatttgaagtggtcagtgatggtttgaacattttttgcaggatgagtgaaaatgcactggattatatttgggatttttgtttttggaattgtctgttttaatcacagccttaattcacaattggcaaaggcagtttactcaaaggactgggctaaatattctgtaattatgcatttttgataggaaaatgaaatttttgcaaacagacattttctttttttttggctggagtgcagtggggcatggtcttggctcactgcagcgttgaccacctgggctcaagtgatactcccgcctcagccacccaagtagctggcactacgggcacacgccaccatgcccagctaatttttttgtatttttagtagagatggggttttgccatgctgcccaggctggtctcaactcctcagctcaagcaatctgcctgcgtgagcctcccaaagtggtggaattacaggcgtgggccactgcgcctggcccagacagacattttctgaaacacaactggcaatgagctgtttttacattttgaaagtgattcttcacttcctagttcttaattatagtatacctattaagatctgtaagatcctgaagacataagatcatgaagccatataagaatgaggattgaaagttgagcaaaattttcgggattttgggaaacattcttagctgtgctatctgcctaaaattattccttattacttctctcctttgacagacttcaagttttcttcatagccctttcaaagttttttgagccatccagagtaaaatcatttctaaatgatagttctgtatatctccaactcgtcttaagtgtatttgcctgtgtgcaacgtattgctagactatgaactcctcagcatggctgctggataacttaattgtcctgagttaatagccttcaaaggacaaatcggtttctttgcagatagcttcgtaaaacttcacatggagtttattttatcatatttcccttttttatttctgctcctcctttaattgcccatcttgcttcagagactgacatttcagggtggatattaattaaagcattaattttgttttttggtatatttctatccctagtatttctatcttactgctaaaatacaggaaaagtgccgtatttttaatgcatttagtggttttctttggtgttatctgttccatttttctttttcatacattgaagtgtgtctccttttcaaccaaaataatgaaatagtggagaccatgaaattgttgtgcctggctaattggcaaattaatttaccaatataataagtgtagcgccttgtttgaataccctttttgagaaggtatgatgagaatgggcaagggtgtcagcatctcttcttcttaataattaattgttttcagttttggttcacgaagaatgcttagttaatctgtaatgttgcctagagctgtatttatctgtttttatttatactagtgtagtaaagctgcatatcattacagtaaaaacgactactgtgatgagttaatcagaaaatctattaaaatctatatgacaatgaaaaaaaaaaaaaaaaa

SEQ ID NO: 11 - DNA, 3006 bp, Homo sapiens
gcaggctgctgtctcacagagcgagaaggtgtcaggagcagcccagttgtgtctctctctctacctctgtgaagggcgcgaatgggcagagcagaacttctagaagggaagatgagcacccaggatccctcagatctgtggagcagatccgatggagaggctgagctgctccaggacttggggtggtatcacggcaacctcacacgccatgctgctgaagctcttctcctctcaaatggatgtgacggcagctaccttctgagggacagcaatgagaccaccgggctgtactctctctctgtgagggccaaagattctgttaaacactttcatgttgaatatactggatattcatttaaatttggctttaatgaattctcatctttgaaggattttgtcaagcattttgcaaatcagcctttgattggaagcgagacaggcactctgatggttctaaaacatccctacccaagaaaagtggaagaaccctccatttatgaatctgtccgggttcacacagcaatgcagacaggaagaacagaagatgaccttgtgcccacagcaccttctctgggcaccaaagaaggttacctcaccaaacagggaggcctggtcaagacctggaaaacaagatggtttactctgcacaggaatgaactgaaatacttcaaagaccagatgtcaccagaaccaattcggatcctagacctaacagaatgttcagctgtacaattcgattattcacaagaaagggtaaactgtttttgtttggtatttccattcaggacattttatctctgtgcaaagaccggagtagaagctgatgagtggatcaagatattacgctggaaattggtcaaggacaaaagctgatttattttgtctgctctctgtatatctcccgaggagaagactgatcacaaataagaaaacagctcaaccaaggggaaggcacgatccgatctcggtcgttcatctttaaatagatctttcttgccaaggaatgctctggcccaggagcaaggtggaatgtttccctgacgctgtgatctgcagcaggcttcaaatgaaaaccgactaaggattttctttcaaaaacaaatcagaagcagatgctgattgggacccatataccacgttgctgactcacgttgctgcccttccatgatgttgccatctccttgagaacactgaagcaatcaccattctgatagaaagtgcttaaaccaccactcttaggtctgctcactcttagaacacacaatggaagaggaagggtttttgttttcactcattgtggtccccaagcctattgacactagttgcctagagtcccactgtgagtcatggtcagcctgtctgacatccaggttgtgctattaaccaagaaggaaacagatacttggaggcttagatgacttctgcaggatttatattcagatagaaaacatcaaatattttcaggggagaggtttttttttttaatttttccccctttatacaaaaaaaaaagaacatttccaaaactaaaatagaaaatgcttgtggcatttattttctctttttaaaaggttcagaaatttggcaggtcctttgcttctaatgacaaaactgtgagagctagatgtcctatgggcaattaggtagtataataaaggtaaatgaaggtacaatttttaaaccattattttcaccctgttggggtaaatgttttaaagagtgagaaaacataaattgagaaagggtgataaagtaatagataacttttagtttaataataattattgttattatactactaataatagagcacttgtaagcactaagttatctttatccaacatttctccaaatggactgaaagaaacttttcaaggacagtgtattataacaatccctttcccagaattagttgtatagggttggcccaagagatgtaagaaaaatctcgcattgctccctaagcaccctgggccttattaaagagcaacttctatttccagtcgggggagtaacactaaagctacaagaaatatgtaataatgataggtaataatgtgttccaaagctttttcaaactagaataaggaggcaaatagaagaatgagatactgatgtccacagttcattggcagaatctaaccccttctgttatcttttttaatactatttttgtttagatagaagtttcaaagaagataaaaatgcttgaagagcctgagagtaaaaagattatgctgcaaagctatgatataaactgctcttgcagtccaaagggatacctgattaaagaagtttcttatttaaacatctcagacgcaaaaattacattaaatttttgtatatttcaacaacattttaaatgtattttgttatgtttgtattatataggataaagcaaatgtcaagttaaaatgtattgtgttgtttgtaaagtaagaagttactggccaggagcggcggctcatgcctgtaatcccaggactttggtaggccaagacaagcagatcacttgaggtcaggagttcaacatcagcctggccaacatgatgaaaccttgtctttactaaaaatacaaaaattagctgggcatggtggcaggcgcctgtaatcccagctactcaggaggctgaggcaggagaattgcttgaacccgggaggtggaggttgcagtgaaccaagatcgcggcgctgcactctagcctgggtgacagagtcagactccgtcccaaaaaaacaaacaaacaaaacaaaacaaaaaaaaacagaagttacaaatgaatactcacggatatgtatagttttatgtttgttttcttagaaacaaatgtgtttctttgggtgggtaatattgtgttttactatgtttaccttttataaaacataacctgtttatttatattctttggctttgtttattaaaaagcatgattttgctgtgcatgtaccattttgctattaaaatttatttttaatatttgtaacttgaaaaaaaaaaaaaaaaaa

SEQ ID NO: 12 - DNA, 1861 bp, Homo sapiens
agcctactcggtccggggttgcgaactgtaaggtctgagttgctgcggcgcaggcagcggagaccaagcagggatcttaacagggtttagcgccacgcgggccagggccgaggccggagctgggaggggcgcgcccgggaaggggcggagctgcggcggtggcgccaaatcgcaaatatggcgccggagcggctgcggagccgggcgctctccgccttcaagttgcggggcttgctgctccgtggtgaagctattaagtacctcacagaagctcttcagtctatcagtgaattagagcttgaagataaactggaaaagataattaatgcagttgagaagcaacccttgtcatcaaacatgattgaacgatctgtggtggaagcagcagtccaggaatgcagtcagtctgttgatgaaactatagagcacgttttcaatatcataggagcatttgatattccacgctttgtgtacaattcagaaagaaaaaaatttcttcctctgttaatgaccaaccaccctgcaccaaatttatttggaacaccaagagataaagcagagatgtttcgtgagcgatataccattttgcaccagaggacccacaggcatgaattatttactcctccggtgataggttctcaccctgatgaaagcggaagcaaattccagcttaaaacaatagaaaccttattgggtagtacaaccaaaatcggagatgcgattgttcttggaatgataacgcagttaaaagagggaaaattttttctggaagatcctactggaacagtccaactagaccttagtaaagctcagttccatagtggtttatacacagaggcatgctttgtcttagcagaaggttggtttgaagatcaagtgtttcatgtcaatgcctttggatttccacccactgagccctctagtactactagggcatactatggaaatattaatttttttggaggtccttctaatacatctgtgaagacttctgcaaaactaaaacagctagaagaggagaataaagatgctatgtttgtgtttttatctgatgtttggttggaccaggtggaagtattggaaaaacttcgcataatgtttgctggttattcaccagcacctccaacctgctttattctgtgtggtaatttttcatctgcaccatatggaaaaaatcaagttcaagctttgaaagattccctaaaaactttggcagatataatatgtgaatacccagatattcaccaaagtagtcgttttgtgtttgtacctggtccagaggatcctggatttggttccatcttaccaaggccaccacttgctgaaagcatcactaatgaattcagacaaagggtaccattttcagtttttactactaatccttgcagaattcagtactgtacacaggaaattactgtcttccgtgaagacttagtaaataaaatgtgcagaaactgcgtccgttttcctagcagcaatttggctattcctaatcactttgtaaagactatcttatcccaaggacatctgactcccctacctctttatgtctgcccagtgtattgggcatatgactatgctttgagagtgtatcctgtgcccgatctacttgtcattgcagacaaatatgatcctttcactacgacaaataccgaatgcctctgcataaaccctggctcttttccaagaagtggattttcattcaaagttttttatccttctaataagacagtagaagatagcaaacttcaaggcttttgagattcttaaagatcatctgaagaaaattcatcagttttctgcttaactctatatcttatgtgattctgatattacaataaaattatggtaaactttagga

SEQ ID NO: 13 - DNA, 1307 bp, Homo sapiens
acttatctgcagacttgtaggcagcaactcaccctcactcagaggtcttctggttctggaaacaactctagctcagccttctccaccatgagcctcagacttgataccaccccttcctgtaacagtgcgagaccacttcatgccttgcaggtgctgctgcttctgtcattgctgctgactgctctggcttcctccaccaaaggacaaactaagagaaacttggcgaaaggcaaagaggaaagtctagacagtgacttgtatgctgaactccgctgcatgtgtataaagacaacctctggaattcatcccaaaaacatccaaagtttggaagtgatcgggaaaggaacccattgcaaccaagtcgaagtgatagccacactgaaggatgggaggaaaatctgcctggacccagatgctcccagaatcaagaaaattgtacagaaaaaattggcaggtgatgaatctgctgattaatttgttctgtttctgccaaacttctttaactcccaggaagggtagaattttgaaaccttgattttctagagttctcatttattcaggatacctattcttactgtattaaaatttggatatgtgtttcattctgtctcaaaaatcacattttattctgagaaggttggttaaaagatggcagaaagaagatgaaaataaataagcctggtttcaaccctctaattcttgcctaaacattggactgtactttgcatttttttctttaaaaatttctattctaacacaacttggttgatttttcctggtctactttatggttattagacatactcatgggtattattagatttcataatggtcaatgataataggaattacatggagcccaacagagaatatttgctcaatacatttttgttaatatatttaggaacttaatggagtctctcagtgtcttagtcctaggatgtcttatttaaaatactccctgaaagtttattctgatgtttattttagccatcaaacactaaaataataaattggtgaatatgaatcttataaactgtggttagctggtttaaagtgaatatatttgccactagtagaacaaaaatagatgatgaaaatgaattaacatatctacatagttataattctatcattagaatgagccttataaataagtacaatataggacttcaaccttactagactcctaattctaaattctacttttttcatcaacagaactttcattcattttttaaaccctaaaacttatacccacactattcttacaaaaatattcacatgaaataaaaatttgctattga

SEQ ID NO: 14 - DNA, 1922 bp, Homo sapiens
gtgcgcggccccgcgcggcaacgcaggggcggaaccgcatgactggcagtggcatcagcgatggcggctgcgtcggggtcggttctgcagcgctgtatcgtgtcgccggcagggaggcatagcgcctctctgatcttcctgcatggctcaggtgattctggacaaggattaagaatgtggatcaagcaggttttaaatcaagatttaacattccaacacataaaaattatttatccaacagctcctcccagatcatatactcctatgaaaggaggaatctccaatgtatggtttgacagatttaaaataaccaatgactgcccagaacaccttgaatcaattgatgtcatgtgtcaagtgcttactgatttgattgatgaagaagtaaaaagtggcatcaagaagaacaggatattaataggaggattctctatgggaggatgcatggcaatacatttagcatatagaaatcatcaagatgtggcaggagtatttgctctttctagttttctgaataaagcatctgctgtttaccaggctcttcagaagagtaatggtgtacttcctgaattatttcagtgtcatggtactgcagatgagttagttcttcattcttgggcagaagagacaaactcaatgttaaaatctctaggagtgaccacgaagtttcatagttttccaaatgtttaccatgagctaagcaaaactgagttagacatattgaagttatggattcttacaaagctgccaggagaaatggaaaaacaaaaatgaatgaatcaagagtgatttgttaatgtaagtgtaatgtctttgtgaaaagtgatttttactgccaaattataatgataattaaaatattaagaaataacactttcctgacttttttattattaaaatgcttatcactgtagacagtagctaatcttattaatgaaaaacaatagacaaacatctgtgcataatttttcagacacaattctgtaaatatttggaaaccttttaagtatttaaacttttaaatttttgaaataaagtattctaaactaatataaataaggacaatgaaaaaacatgaaaggacttagcataatgttattttatcttttctacaactttgtttaaattacctttccaaagatatttgtgtttatgtaattttccacggaataacattaatactctaggtttataaaccggtttcacattatttcatttgatcatcacaagagctttgtgaagtaagccgagaagttgttactggtatttaataatagcaatagaggagttaaagactttcccacagcttgcaggtcaagacaagaaattcaggtctcctaattctcagtggagctctatttctgttaacccaaattgctgctctgttttaggtctcaatttcatctgtaaaatgatactaatagtacttatcccattggatttttgttgagatttaaataaatagccaaaagccaatacataataaacactcaataaagattaaccataaggagagtcatgatctggttccaggaatacattgttagatgactgaaaaattgtattacttcaatgaaaatactataaataataacattttcatatattagttggttctcatgcatacataatctaattttatttgatcctcacaactgtttaagttttattaaatatacattatccctatttgtataaatagaatcatacaatacctgcctgctttcattcaacaaaattatcatgagatttttccatgttgtgtacatcaatagttcatctattttattgctcagtaatattccattgtgtggatgtatcactatttgtttacacattcaccactgatatataagttgcttccagtgtgaggctgttttaaataaagctgctatgaatattcatgtaagaaaaaaaaaaaa

SEQ ID NO: 15 - DNA, 2269 bp, Homo sapiens
cgcagccccggttcctgcccgcacctctccctccacacctccccgcaagctgagggagccggctccggcctcggccagcccaggaaggcgctcccacagcgcagtggtgggctgaagggctcctcaagtgccgccaaagtgggagcccaggcagaggaggcgccgagagcgagggagggctgtgaggactgccagcacgctgtcacctctcaatagcagcccaaacagattaagacatgggaggtgaaagacaacttgagtggttaaattactgtcatgcaaagcgactagatggttcagctgattgcacctttagaagttatgtggaacgaggcagcagatcttaagccccttgctctgtcacgcaggctggaatgcagtggtggaatcatggctcactacagccctgacctcctgggcccagagatggagtctcgctattttgcccaggttggtcttgaacacctggcttcaagcagtcctcctgcttttggcttcttgaagtgcttggattacagtatttcagttttatgctctgcaacaagtttggccatgttggaggacaatccaaaggtcagcaagttggctactggcgattggatgctcactctgaagccaaagtctattactgtgcccgtggaaatccccagctcccctctggattgtcagtggctgctatgcagcaggtgcagcctggtctctcactgagtctctactccacaaaggcaacgactggccaaggcagtggctggctctgggttacacaagtgcagacactcaactaagtgagctggaagacccaggagaaggcggaggctcaggtgcccacatgatcagcacagccagggtacctgctgacaagcctgtacgcatcgcctttagcctcaatgacgcctcagatgatacaccccctgaagactccattcctttggtctttccagaattagaccagcagctacagcccctgccgccttgtcatgactccgaggaatccatggaggtgttcaaacagcactgccaaatagcagaagaataccatgaggtcaaaaaggaaatcaccctgcttgagcaaaggaagaaggagctcattgccaagttagatcaggcagaaaaggagaaggtggatgctgctgagctggttcgggaattcgaggctctgacggaggagaatcggacgttgaggttggcccagtctcaatgtgtggaacaactggagaaacttcgaatacagtatcagaagaggcagggctcgtcctaactttaaatttttcagtgtgagcatacgaggctgatgactgccctgtgctggccaaaagatttttattttaaatgaatagtgagtcagatctattgcttctctgtattacccacatgacaactgtctataatgagtttactgcttgccagcttctagcttgagagaagggatattttaaatgagatcattaacgtgaaactattactagtatatgtttttggagatcagaattcttttccaaagatatatgtttttttcttttttaggaagatatgatcatgctgtacaacagggtagaaaatgataaaaatagactattgactgacccagctaagaatcgtgggctgagcagagttaaaccatgggacaaacccataacatgttcaccatagtttcacgtatgtgtatttttaaatttcatgcctttaatatttcaaatatgctcaaatttaaactgtcagaaacttctgtgcatgtatttatatttgccagagtataaacttttatactctgatttttatccttcaatgattgattatactaagaataaatggtcacatatcctaaaagcttcttcatgaaattattagcagaaaccatgtttgtaaccaaagcacatttgccaatgctaactggctgttgtaataataaacagataaggctgcatttgcttcatgccatgtgacctcacagtaaacatctctgcctttgcctgtgtgtgttctgggggaggggggacatggaaaaatattgtttggacattacttgggtgagtgcccatgaaaacatcagtgaacttgtaactattgttttgttttggatttaaggagatgttttagatcagtaacagctaataggaatatgcgagtaaattcagaattgaaacaatttctccttgttctacctatcaccacattttctcaaattgaactctttgttatatgtccatttctattcatgtaacttctttttcattaaacatggatcaaaactgacaaaaaaaaaaaaaaa

SEQ ID NO: 16 - DNA, 7091 bp, Homo sapiens
gctacccacttccgccccctccccctgccattggaactagctgagccgaactagttgcggccaccgagcagccggctctcggcacctcctcctccgcctccctgtctcctgttccattcgcctttcctcttctttcctggcccacgccgctccgaggcctcgcgaccgccgagcctgcagcctgccccgcggccaacatgagcttcttgttgagttctcagcctgaagttgactggaactttcagttaacaagtatttatcgaatacctgatctgtagtgttggacttagacctatggaaggagctactgatgtgaatgaaagtggtagtcgctcttctaaaacttttaaaccaaagaagaacattccagagggttctcaccagtatgagctcttaaaacacgcagaagccacacttggcagtggcaaccttcggatggctgtcatgcttcctgaaggggaagatctcaatgaatgggttgcagttaacactgtggatttcttcaatcagatcaacatgctttatggaactatcacagacttctgtacagaagagagttgtccagtgatgtcagctggcccaaaatatgagtatcattgggcagatggaacgaacataaagaaacctattaagtgctctgcaccaaagtatattgattacttgatgacttgggttcaggaccagttggatgatgagacgttatttccatcaaaaattggtgtcccgttcccaaagaatttcatgtctgtggcaaaaactatactcaaacgcctctttagggtttatgctcacatttatcatcagcattttgaccctgtgatccagcttcaggaggaagcacatctaaatacatctttcaagcactttattttttttgtccaggaattcaaccttattgatagaagagaacttgcaccactccaagaactgattgaaaaactcacctcaaaagacagataaaaggatgcagagctgtgcaaattgttcctcaaatgaagcagtgtggagtgtattggggattttgttatattttgtttttatctggattgtttttgtcctaggtttgggggcgggggcttgtttgggttcctttttctttattctgattatgtgaaaccatattctattgctaggggaagccaagaaccattctctatacacttgataagggtaaatttatcttagtgtttttaaacttggttttggttacttgaggagttttttaataatattgtgtgctgcaagaaagtgcttgttgattgaactgccgatggattggtttctgtgtggtataaattgtggcccatttatgaagtccccaaaagagttatgtttttaagtgccttggcaggctcacttctgaggtgcaaaacatagatatagaactgaacagggcttgaaacaatattaggattactacccagggcacttactggtgcatgttgtaacatatctatgataaaagccatagtttacctaaaatggtgatttccagcctttactgctttgaagaaacagaatttgtaaaggtatgcatgtagaacataaaaaatatttcttaattattttttatattgatggtaatatattacgttcaacaatgcttaaagctctacaagcaggtcttttcccacctcttgatatctgtgatactgaaacttgaggatgttgaaatgtattacattttggcttctttctacatgttaactgcactgtagatgtaaaaattcaggttatatataggattgccatcttcagaggtgatgctgaactgtgaggtttcctagtaattgccaaatgagccgtaagtctgcagaattcccttctactttgaagagaaggggataggaatgtatatttggctgggggcatggagatgttcgtatgtatgaggagttagggatggggagtcaagttctagaaagttttgtctgaaaacctttgaatagaatggcatgaagattttaatcaattacttataaacaaagtcttagagacttccttttaggaatcaacttccatgagaagttaaaaataaattattaattttaggtacagacattaaacatggaatttaaggactgttgggggaaattgatcacttcttagcatttccattcagtgaatggagctgatgtttgcctgtcattttaagatgataccataccttctttggttattataggtccagtttgaagcattctgacttctggtttttccaccctgaaaggaaatgtttttctttgcagcagtattagataatgaaaaatgctaattcagtagttattaacttctaaattttattcgccatgactttctagtgaattattaccataaataacaatttcagaaacttagtttttagaataaatattaatttttccacttcagttttattctagaaaataccctttttagaaatccagttttagttttgtcattttcgataaatctttcttcagttagaaatatatatccttccttcagttgaaacatatacctttttcacatctaggaagaaatgcttgctctgaaatagtatagattaaaaacactcagtagaaaagaatctaaaattaaatgaatttgttttgccattaaagtagagcagtgatacaatttaatgccattacaattatgttgactagaaactgcctttttctccacttcatttctagcaattatttaccaagtaccaacagtagaagtaacaggaaagcctggcagagttaaatatcttggacatttattggtaaagcttatttataaactgcagtcagagctagttaatttccttaaatctttttgtattcagatagataatatgaatcattatgggttgattcagaaataaaatttgtgaggtgattttgaatcttgtccatataggaaaatgaagcacagaattactcagtcttccatattgtatttgacttcatatcaatctagtaaaaaaggagttgcaatagccaagtatagagagaatagtgaaaaattaatcttgccctttcaagccttatacagtagtacactgtacttgtttttagtagtaagacctactttcccactatatgtagatagtttgttttcactgtgccagaatctcaggtgcctgcttagagtatttctttaatcacagtcactgggaagtaaggagatgtatatatgtgtatatatggtaacaaagcatagcagttctctaggggagaggcctggcattgcacatggtgttacatggctacaagtaaggaaaaaatcagaaagtgaaagaactgatgtaataaaaggttgatttggttggttcccatgaaagttagtaagatgcccttttaaatataaggatcagtgctttgttctgcagcagagtttgctgataaatgtctgttggattctttttggatttctttaattaatttgtaagtaaccaagataattattttcccccttgctctctatattaatacgtagctataaagcaacagttggttttcttatcctttgataaaagcatcccataaaatataaagtagtaagttaacatagtattattgtcacacacaatgctttttttggttaaatgttgatacgaagcaatgttttggaattactttaattgatggagtagtggtggtagagagaaattaataacaaaaagagtgaaaatattttaattagcagtagatggtgctactggctttcatttgctgacttgattattccctttctcttaaaaaccatggcattagactgcactaaattaacaagcatgttagttgctggtagaggttttggaggttaatttaccttaaattggaagacttttaattgcagtctctttctaccttccctctgttagtcatttgtaaattctaaatggtcaccataaaatgtattaggtaggagaagatacgttttatgtataatatatctcagactgagttactgcctgtcttatcaggatggataaaacactacagtctcttatcaggaaatagagatgatgtggatatttatatattacatatataaccaccagactccattttatatattagcattttccttgcttatgggaaaatagcaaaacaacatttcatttatacttttgtttacccctctctgagacaggttttgataaccactgaaatggtagaatatgtgagatacaaatattgagttgtagaactttctttttaaggtgaataagtcatgccttaacatccaaataagagttcatcttcagagtggttcttttgggagcactgtttattccagctatactgcaaaagtataatgtttttggaactgttctagagcataccatgaaaagcagtttgttattatgcaggaaaatcagtttcatcattttagttacactaaacacttttggcagcttaatatgacctttttaaattttttttattttttttatttttatttctttaagatggagtcttgctctgttgcccgggctggagtacaatggcatgatctcagctcactgcaacctccacctcctgggttcaagcatttctcctgcctcagcctcccaagtagctgggattacaggcagcaccacacctggctaattttcatatttttagtagagatggggtttcaacatattggccaggctggtctcaaactcctgacctcaagtgatccgccctccccagcctcccaaagtgctgggattacaggtgtgagccaccacagccagccagtatgacctatcttaatcatcagctcaactgtaatttaaatttggctgttctctggagctaaaccattagggaagttcaaaggaatgtgccatgatttccgaatttgcacaagagaatgttttaagcattggtagcataattgaataaaagaatagtttcctgatgtcactattttgaagtggaaattatcacttggatgtggaggttttactttttaaaaacattcagcttaattaccttaccttaattaccttagttagatatactaatggaaaaaaaccaagtcctttctctagaacttgttttctatttttgttccttttcatgaaaacttctcaatttaattttaactactgtaggatagtattgattgaatggatactatggaaaagtggatccaatatttaagatagaagtagtttaaggagacaacagcctttactgccatttttttttaaatgttttcactcagatgaacaatttgactttaataaaagactggagatttttgtacaaagaaataggaataagtttcatatactaattatgctgagttttaagcctacatatcacaaaatatttagaattgtataaccttttcatatatttataacttttaatgtctttttaaaagatgtgggaccaaaaatatatttataatttggaaatgtgactgcataccaataagaaaacttaccttattttgaaatttatctgggatattaaagaatctaccaattcttaaaaacacagatttatactttaagcttattttaaaattaaagaatatataccaattcttagaaacactttaaggactactcttaaataacttaaatatcagagttttgttgtaatattaaaatttaccgtggaaatcactgttgttcagctatcaccttaattgtgtatgatatgataaatgtttagcagtaaagctatcttaagatttaatggaaaagtttaatttgaagatgtaacaaaaattctgaccacagttgattctgaatttttaaggctttcctaataggctgatcacagagaataatccattttgaaggtataaaactgcactgtatgtctgtcacttgtagctgaactgattcacattttgacaaaagagagaaaatacaaaaatgagttttgcaaatgtaataactttttctgcatatagaactaaataattgaaaaatatgggctatagttctcaaaggtagatagtaaaatcactggctttttccagctgtatgtttttccactgtgcgtgtacacacacactggaaaataattaggctgattttgcaggtcttcattgttagagattctgaagtatttactgtcaattcataggtttcagtttatttaggaaattagtgtttgacagctttttttaaattatttcactgaagctgagattattagtgatacaaagttaaaatttcaatatttaatttctctatatattattaatattaaattgttttttacttataaattcatgttctcatctgatttaatattaaatttgtataggtgggcgtttcttaccattttgcacaagtttttgtttttctgaaatacttaattgtgcaggttgtaaaaaagattagtgcattttcattttaaggatgctttgctccttaaattgttcgacagaaatgactttttagggaaagtagtttttttggagctactaacttgtatttattattgtacatgcataaccagggtggtgagggcactaatcttgtaggaaacacttacttgatgttttatttgaacttttcctataggtttaacttttactgcatagaattaacactaggaacagtgtcatgaaatctgggttgaaggagaatacagtatatatgagaacacttaaagttcaaatagaaatcatttctgaagacaaaagcagaggaatattgtcagtgccaagtaatggaagaataagggcggcatttacactgtgcaagtattgagaagagtgcataaagacagggaactactctcatggagacagtttctctcttataatcaagtaactagaaggggaaaaatcatctaagttatgaaatccaacataggcgctatattacaaactgtgccggattatgcaaattgtagttgttactgatcaaagtttaattgcttcatttttgtttaaaaagggatactgatgtcagaaaatctgtaatatgttttattcaaaagatgtaaataatgtatacagacttgtatgtgatgggatgggaaatatttaaattctaggtgtttttttttttttaaagaagaaactcaatgtttataagaaaaaaatgaataaatagttacgtttggccatgaatcctgaaaaaaaaaaaaaaa

SEQ ID NO: 17 - DNA, 7003 bp, Homo sapiens
actcgcagtcctgacgggcaggggctgcggaccgcccggccttggacccatccggagccacaggttggaggagataagtagctgtccccgtgctcatcgccctgtggagcagatcctgtctccttgctgacggtggagcccgggagttccagggcttgggaaggggaaggaaacctctctgaaatctgacacctgctctcccggcaaggaaacttcgcaggctgaccgaccaagaccatcactatgaccgatggagactatgattatctgatcaaactcctggccctcggggattcaggggtggggaagacaacatttctttatagatacacagataataaattcaatcccaaattcatcactacagtaggaatagactttcgggaaaaacgtgtggtttataatgcacaaggaccgaatggatcttcagggaaagcatttaaagtgcatcttcagctttgggacactgcgggacaagagcggttccggagtctcaccactgcatttttcagagacgccatgggcttcttattaatgtttgacctcaccagtcaacagagcttcttaaatgtcagaaactggatgagccaactgcaagcaaatgcttattgtgaaaatccagatatagtattaattggcaacaaggcagacctaccagatcagagggaagtcaatgaacggcaagctcgggaactggctgacaaatatggcataccatattttgaaacaagtgcagcaactggacagaatgtggagaaagctgtagaaacccttttggacttaatcatgaagcgaatggaacagtgtgtggagaagacacaaatccctgatactgtcaatggtggaaattctggaaacttggatggggaaaagccaccagagaagaaatgtatctgctagactctacatagaaactgaacatcaagaaccccaccaaaatattacttttaaaaacaatgacaaaccacacaattgttgttgagtaaaccacgcacaatggcatgtctttctttttctgccagaaaatctattttaagaaaccagaatagtcaacagtgttcaaaagaattgactagttatccctgaggccctttcaaacatgatcaaagatttcccaatgtgatctcatcatcatggatactcaatttgttttttcttatagagaaaatgagtatataagacaatatacaagaagaaatatcagtgagttttaaatcagaacaagttacctgtcacattgaagaaaagggtaggcactaaagggagaacacagaaagaagaatttctaaaatattggatttacttcttatattgagtcagatgcatacttttagatttgcattggggaaaatgtactagctaaaaatggatacacaatgaagaattctatttggctaattaagaatgatatactatgtacacccaataagctgtactagaatgaataaattactgataaggttacaaataggtaaatgtcacacttctgttaaaatgcaggaggtagtgtcataatgccgtctttatattcttaataaatagcactttgacaagaacaggactgtaaatgatgaagtacaagacaaataccctgggaaaaaaaatgaaagtatgagaaattggcatttctacagctgaaattcaatgtatctgttagagatgtctggaagggttacttagccaaattttactcaagccaattaggagctgatattatcagttggaattaagagaactccagaggtttccatttcaaacaaaattttagaaattggtttggtgttcagcttcacatttcattttttcttagcacatgttgataaaatagtcacaaggagaaattaccagttacggtttattaaatctcttttaaaatgcagtcaaggaaaactagccttgaattttttttagataaaataagatggtgatatgaaacaaaaagtggcaattattgcaggtttccttttagtttacaaaagtactggaaactaaatcatatttcttccctccaaatttcacccattcctgactttgaatcaattgcagaaatgcaggtgtgttactttgttgatcaataactttggaacaattatggatcaattctatggtcactctgaattttcatgtcattaatcacataaaaattgataatacctcattctgtattacaatatgattttattttgccaaaggcaagacacctatagttgagctgtattttgggggattgggtgaggaaggacttctgatcttatctcaacaaaaaactggccagtatttttgttaatgtaaagcttccttttctttctaaaaaatagtaacaaaattatttttcattggcctattctgttcttgtgtctaaactaacattacattaatttttaatcttagtttctgataaacacaagccattcctatcaaaatattatttatttcagtcaattttaccaaataacaaagacaatatattttcgtttttttttattatgagcatatgattttttgacaggctgtttcctcgtcgtatagattttttccaatcaaacctactttttccatactctgtgcatattttttgtgaagttatacacattgaagaccctaaaaatcccagtccatcattcagcttacctctgcgaacttctatctggtattgaatcagtttcagaaacacagacagatccaaggaaatgtctctttataatgttcttaggatggactagacccataaatgtgccatgaatcaaaatattaataatttgaaagctttcatgctgttagcccctgatgaaattctcagcattaactggccagctcctctgatttctgcagcatcgcaacaggttcgaagatgggttgtggctgggtattccctcccatggtgtttcctctgggatgctcttcattatctcaatgcctgtgccatgaagatagaaaactgtaagctaacatttaagatgtttcttctggaaggaaagtgagcaggaacaagttatattgccactgctgtggcaaattttggtgaacttttggggtcattatatcaattttttctttggattcaaattgtaatgtcccctgcatttccttaatagggaatgtgaaacctttataaaactctaaaagtattctgttttgatatgtctttttgtttctattcattttcagttatatgattgatttacttatgccaagattctgtcactgtcagttatttaatgagtgttttttcagggtctgttttaagatcattatttgatagctgtagcatgaagcagaggttgatgatgcccataattgcaagactattcctgtaaaaataacaattattgggtaataacttcaagaggaatgagaagtgacaaaattgatttaaaatattgttctacttataaataaatgcttgatataaaaaattttctccataaagtttgacatctgaccccagattctatgtaatcattattagaaattccttctctcattatttcaggattagtagttctgtgtaattcattttacaatttcaaattgttctggtgccataaagtatacagactactttaaagatttccaaatcccctaatttaccccacaacagcatgtaattttagccaagatatgtcctgttactaagtatctcccaatgctttagtaaaacgtatttaggagaaatgttgaaaatgtacatgaagctcctttctgatatagaaaccatttctggagtatttacactggtttgatgtttacattgctctaactcggtgcctcagatacctctgtgaccaaatttgtctccaaccacatagctcatttcctataatgttatatcataggaagccctcacagagacactaacacagctaaagatcttctgatattatcagcaagggatgcaaggactttattggaatctggagagtttaactgccttctcttggtctcctcacttacttcttatgaagttggcattacctgagactcttagctgtgattaggtacaagcttaccttttagggtagaaaaagaaagatcatttgaaaaatgtatctaaaataatccagagaacataatgtttgtcttggtctgataatgataagaagtcaaggattggcagagaaaatactaaacgccaagagttgagcctgtgggtctctccataagagttttaaaactcttgccagttaccactttatccaatttgctatcattttcgtattatcagctatcgccctgtaaaatattcaaaactagctatttctaaagtaaacattttatctgttacttttaaccagataggtgtctttgtcatccttctactataaattgttctttgccaacctgtacaggtagatgaaccaggcgagagttttaatcagccttttcttgtcccctttgtaagaaagagatgcttgccatagagaaggacatgagtacattaaaaataatttaatagccacaatatgatgttctttaagctgcaaattgagtacactgggaatcaacaaatttgatgaagcctgtctgtctcttcaccagtggagtgagtgcagcagttagaaagagaagcaatattgtgcaactggtgcagtggtgagttaatcatagtgtataaccttgtgttcatgaaacaggttgttcattgttctgcatctctcttcatttaaaaaggatacacaattctttcctcattgcatattacaccaaacgtttgagggaaaaatcctcattcgtaaaggattttggatgtataatctaaaactcaacaataaagaaataatattccaagtctctggtttcctaagatacataataactgtttataaagaaggtctaagagctgatatttgccaaagtgatagaagagttgttttttcctctctactaccaagctttaagacattaaaagaagtctagtgtatttgaatattttagagaaagctttatcattttttaagatgccaagatgctgcctacgtttgcaaaagttgtctaagaattcaccatgagctatattttcttctggatctttgaccaaggtgatgtcagcttatttctggggaaggtgttgagctcttatacatgaaaatggatataggctattctctgggatgagtgtcatttcaatgctttataaatccatgaagctgcttgtctcataaagtagaactgatacaaattttggttggatatatagagaattttataaatgtattgccttagaatttctgggtggagacccaactacaatgacattgtcatgccagaactataaagataattagagttaaaagttgtttaaattgtgcccttaaatacagcagaacctggagaaggtcatacttcaaaggtcgattttgagtccgaataaagaaagacctagtaacagatagtttttttttgttcattttcttctaccaagtagaggtttatgccctcagaactaaactagtaaaaatatctgaacaaaaaacctttcgttgttggcataaaaatgtgatacacttagagacattttgtttattgcatataaatctaatttttccataaattagatttatgatattttcataaagcacttgattagtttttcaaggcgtaccatcacaaagatgctttcctgcagagttctttgtatcaacagcctatggttgagatgttttctcatttcctgtagagagagaataccactaacaaacaaacaaaaactttagtgccaaaatagtggaactattttgtcatcttttgagaaaaaaatatacaaagaagtcatcttttcattaagtggattccctggttcctttccagctggttgtggaagtaatggctaacatccttcagctgactttgtctacaaggattattagcaaattctgtaggagcaagcatgtctgaccttaacttaatggatcccttattcaatcagtggcttctgtctttatgtctgttggcatatcaaaatggtttctgttcctagaaaagtaataacatatgcttatctttattctttttccaggtgattttgttttcaaatgctccttgtgaaaacacctagtgttgtagaaaggaaagtggccagaaagaacaacttgggaccatgagtaggtcattaaatagcttagtgatttatcctcatatagggcttataaaccctgtatgtgtttatatgtgcttcacagagttcgtgtcaggctcaaaggagatatgtataagaaagtggtttgtaaattatgttccatttcataaatagacactattcacaaactaaaatctaataaaaaaccacagttgtaatttaaactgcttgatataaaaagaggtatcatagcagggaaaacacactaattttcatacagtagaggtattgaaaactgaaaatgggaaggcaacttgaagtcattgtatttgattgaaaatgtttaatacatctcattattgacaaaatatgtcatcttgtatttatttcaaggaaaccaatgaattctaggtagtatattacaagttggtcaaaatattccatgtacaaatagggcttctgtgtccatagccttgtaagagatactgattgtatctgaaattattttttaaaaaaataaattatcctgctttagttagtgtgttaaaagtagacgatgttctaatataacactgaagtgcttcattgtatcccaacagtttaccttcaagtaatattatctttatttttaggctaagcacgtttgattattttgtctgtctcctatatagatctgttttgtctagtgctatgaatgtaacttaaaactataaacttgaagtttttattctatatgccccttaatagactgtggttcctgacgcacactgttaggtcattattttgttgtaccaaagttctagtggcttcagaaatcatagcatccaatgattttttggtgtctggctatgaatactatggttgagaattgtattcagtgattgtttctgcacacttttcaaataaaaaatgaatttttatcaatta

SEQ ID NO: 18 - DNA, 2158 bp, Homo sapiens
agttctgcatttctgcagagacagaaagaaacgcagctcttgacttcttttttgtaaacattactgtaagagttgtgataactttttattctactatgtatatgtatggaatagtattaataaatgaactagggaaggatgtaataaattagacatctcttcattttagagagaagatggaaacaacattgcttttcttttctcaaataaatatgtgtgaatcaaaagaaaaaacttttttcaagttaatacatggttcaggaaaagaagaaacaagcaaagaagccaaaatcagagctaaggaaaaaagaaatagactaagtcttcttgtgcagaaacctgagtttcatgaagacacccgctccagtagatctgggcacttggccaaagaaacaagagtctcccctgaagaggcagtgaaatggggtgaatcatttgacaaactgctttcccatagagatggactagaggcttttaccagatttcttaaaactgaattcagtgaagaaaatattgaattttggatagcctgtgaagatttcaagaaaagcaagggacctcaacaaattcaccttaaagcaaaagcaatatatgagaaatttatacagactgatgccccaaaagaggttaaccttgattttcacacaaaagaagtcattacaaacagcatcactcaacctaccctccacagttttgatgctgcacaaagcagagtgtatcagctcatggaacaagacagttatacacgttttctgaaatctgacatctatttagacttgatggaaggaagacctcagagaccaacaaatcttaggagacgatcacgctcatttacctgcaatgaattccaagatgtacaatcagatgttgccatttggttataaagaaaattgattttgctcatttttatgacaaacttatacatctgcttctaacatatcgcatgtttatgttaagatttggtcccatcctttaaactgaaatatgtcatgtgaaattattttaaaaatgtaaaaacaaaactttctgctaacaaaatacatacagtatctgccagtatattctgtaaaaccttctatttgatgtcattccatttataatcagaaaaaaaacttatttcttaatcaaaaggcagtacaaaaaaagtaataatgttttataagattgtagagttaagtaaaagttaagcttttgcaaagttgtcaaaagttcaaacaaaagtctagttgggattttttaccaaagcagcataatatgtgttatataaacataataatactcagatatccaaatgttcagatagcatttttcataatgaatgttctcttttttttggtaatagtgtagaagtgatctggttcttacaatgggagatgaagaacatttattattgggttactactaaccctgtcccaagaatagtaatatcacctctagttataagccagcaacaggaacttttgtgaagacacattcatctctacagaacttcagattaaatataatctagattaatgactgagaataagatccacatttgaactcattcctaagtgaacatggacgtacccagttatacaaagtacttctgttggtcacagaaacatgaccagattttgcatatctccaggtagggaactaagtagactaccttatcaccggctaagaaaacttgctactaaactattaggccatcaatggcttgaataaaaaccagagaaggtttttcccaggacgtctcatgtttggccctttagaattggggtagaaatcagaaatgagatgaggggaagaagcaaggagtctaaggccctagcgatttgggcatctgccacattggttcatattcagaaagtgttatctcattgattatattcttgttaagcaaatctccttaagtaattattattcaaataagattatactcatacatctatatgtcactgttttaaagagatatttaatttttaatgtgtgttacatggtctgtaaatatttgtatttaaaaatgccatgcattaggctttggaaatttaatgttagttgaaatgtaaaatgtgaaaactttagatcatttgtagtaataaatatttttaacttcattcatacagttaagtttatctgacaataaaagctctgactgaaaaaaaaaaaaaaa

SEQ ID NO: 19 - DNA, 5852 bp, Homo sapiens
ttttgccggatgttgttgtatgtccgagagacacgtgaggttctgctacgtcattaccaggcacgcgcaggaaacatggcggcggcgggtgttgtgagcgggaaggtttttggtttcttcttgattcaatcttgataagtagtatgtgtccaggactttatccatactccagtttgttggagtatggtaggagtatgattatatatgaacaagaaggagtatatattcactcatcttgtggaaagaccaatgaccaagacggcttgatttcaggaatattacgtgttttagaaaaggatgccgaagtaatagtggactggagaccattggatgatgcattagattcctctagtattctctatgctagaaaggactccagttcagttgtagaatggactcaggccccaaaagaaagaggtcatcgaggatcagaacatctgaacagttacgaagcagaatgggacatggttaatacagtttcatttaaaaggaaaccacataccaatggagatgctccaagtcatagaaatgggaaaagcaaatggtcattcctgttcagtttgacagacctgaaatcaatcaagcaaaacaaagagggtatgggctggtcctatttggtattctgtctaaaggatgacgtcgttctccctgctctacactttcatcaaggagatagcaaactactgattgaatctcttgaaaaatatgtggtattgtgtgaatctccacaggataaaagaacacttcttgtgaattgtcagaataagagtctttcacagtcttttgaaaatcttcttgatgagccagcatatggtttaatacaaaaaattaaaaaggacccttatacggcaactatgataggattttccaaagtcacaaactacatttttgacagtttgagaggcagcgatccctctacacatcaacgaccaccttcagaaatggcagattttcttagtgatgctattccaggtctaaagataaatcaacaagaagaaccaggatttgaagtcatcacaagaattgatttgggggaacgccctgttgttcaaaggagagaaccggtatcactggaagaatggactaagaacattgattctgaaggaagaattttaaatgtagataatatgaagcagatgatatttagagggggacttagtcatgcattgagaaagcaagcatggaaatttcttctgggttattttccctgggacagtaccaaggaggaaagaacccaattacaaaagcaaaaaactgatgaatacttcagaatgaaactgcagtggaaatccatcagccaggaacaagagaaaagaaattcgaggttaagagattatagaagtcttatcgaaaaagatgttaacagaacagatcgaacaaacaagttttatgaaggccaagataatccagggttgattttacttcatgacattttgatgacctactgtatgtatgattttgatttaggatatgttcaaggaatgagtgatttactttcccctcttttatatgtgatggaaaatgaagtggatgccttttggtgctttgcctcttacatggaccaaatgcatcagaattttgaagaacaaatgcaaggcatgaagacccagctaattcagctgagtaccttacttcgattgttagacagtggattttgcagttacttagaatctcaggactctggatacctttatttttgcttcaggtggcttttaatcagattcaaaagggaatttagttttctagatattcttcgattatgggaggtaatgtggaccgaactaccatgtacaaatttccatcttcttctctgttgtgctattctggaatcagaaaagcagcaaataatggaaaagcattatggcttcaatgaaatacttaagcatatcaatgaattgtccatgaaaattgatgtggaagatatactctgcaaggcagaagcaatttctctacagatggtaaaatgcaaggaattgccacaagcagtctgtgagatccttgggcttcaaggcagtgaagttacaacaccagattcagacgttggtgaagacgaaaatgttgtcatgactccttgtcctacatctgcatttcaaagtaatgccttgcctacactctctgccagtggagccagaaatgacagcccaacacagataccagtgtcctcagatgtctgcagattaacacctgcatgatcactgttcttgcttttttgggaagagacactttgttgcaaccctttttcaagtacttgaaagttgaaaatttgaaatcttggtattgatcatgctttaaggtttatgtaaagaaagtgtactgatgttcttacattaaagctttacaaagatttaaactaattatttttgtagttacttctaccaaatagcctttccttttcgataacattcctcagtatttttatagccaagtacattttattttcttgctgatgaactggaattggataaatattgcaagtggatgagttggaaattatgcactttgaaaaacattcactttgtttaagcttattgggtttcagatttgattaaattaaatgtggaggctttctatagcattctaagctgagaagtagattgttacccagtaatgaaataaaaaataaaaataaaaggatttttttctctattgtttacgacagtactcagcttaaatatttatgctggtcaaatgtgatttaaattggacattttcatcaatgcagtctaatgtgtagataaatatttcaaccataataagtggattggcagtatattttttacattgaacttttcttcacttgtatataaagattatatataagtacttatttatgagtataagaaaggttaggcatattttcattaactgaataaacgacttgatttatataacctggtttatcaaaatttaacatggcttcagtatgagatctttttcaaaactattttcttaaacatttatttcatgagattatgttcaaccctgtacctggtgtaattttaaaattaattgcttgtaacctcactttactaataatgtttattatctttcctaataatgcattaactgattaatcaggtgtttaaatttttataaaatactcttgcaaaaagtttatttgaaaaatttctagatggtctcatgagtttcaaaataataatttttgtgtatgaacaaagctgttgtttttaccatgcagtattgcatgattttaagttatgtggaattaacataactgattttgttttaattgtaagttgttaactcctgtatatatcattaaaataaatctgaagttgaagtagtgtttttagttaaattatacttagaaatagtctgcttttttaaaattttttttcttgagaaagagtcttgctctgttgcccaggctggagtgcagtggcgcagtcctggctcactgcagcctccgccttctgggttcaagcgattctcctgtctcagcctcccgagcagctgggactacaggcttgtgccatcgcgcctgactaatttttgtattttgagtagagatggggtttcaccatgttggccaggctggtctcgaactcttgacctcaagtgatccactcgcttcagcctcccaaagtgctgagattacaggtgtgagccactgtgcccggctaattctttaatagaagaaaaaacatccaagatggacctcaattcatctcttatttttatatgattaaaatgataatctggccgggcgcggtggctcacgcctgtaatcccagcactttgggaggccgaggcgggcggatcacgaggtcaggagatcgagaccatcccggctaaaacggtgaaaccccgtctctactaaaaatacaaaaaattagccgggcgtagtggcgggcgcctgtagtcccagctacttgggaggctgaggcaggagaatggcgtgaacccgggaggcggagcttgcagtgagccgagatcccgccactgcactccagcctgggcgacagagcgagactccgtctcaaaaaaaaaaaaaaaaaaatgataatctgaataagttatggaaatgaaaaccatcctttttataactgaaaaaaaattttcattagcatggaaatgggcacagtgttgccttgaaagatacagttatttgactcagtaaagcagcttattacaactgatgctaatagtatagagaaaaaagttgtgcagttctaaaatggtcctagagattgacttttttcccccaagaaagttagggaacaaaacgaacttttttcctggttgagcattaactgacaatcacgacagtagaaccgttagagtttagtttttaatattatgtgtgttatctttcatcagttaataatgagtaagcctattcagaaaaagaacataaactgatcaaaaactcagcatctccagcctttcatttcctgctattcaggaaattgcttagaacatcttgatgtcctccttgttcttcctggacagtgactttttgggagtttgttcctgctgcgtaatgtgatacccacttcagattttttttttatcaatacatttagtaagttgaacttctgtcaagttttattacaaaattacttgttaaaacaatttttactaaactgcatttctatctagcatatttttgatatggaagtgatagtatagtatagttccaggagaagtcttaaatcagtccacagagtccagttagcaaatactctgtgccattaagattgctaaaatacacagttcaggtaaatttactagtgttttttaaaggtttatttgttttcacaagatgctctgtccacacccttataacatgtaaaatattgtgtgctgtattatgtggtaaagttgttaaaattcagtttctaacattaacttaaaagtacagacaatctaacatgatgatttgacttacaaactttcaactaaatttatgatggctttaaagcagtgcactgaatagaaaccatactttgagtacccatacagccatttttcacttttactacaatattctataaatcacatgagatatttaacactttattataaaataggctttgtgttagatgattttgcccaaatgtaaactaatgtagtgttctgagcatgtttaagttagggtaggctaaactatgtttggtaggttagatgtattaaaagcatttttgattaatgatgtcttcaatttatgatgtgtttattggaacataacctcaatataagttgaaaagcatatgtattttcaattctggcatgaacctatgggaatcttttgcatttaagaacctccccattttaataatttcatgggtctaagattcttcatctgtttataaggaactttagtcttagtgattagagactaaatttttttttgagcagtaagaaaacagccttttgggacagatagtgagtgattcttaggaacttgacattgccaagaaattttatagatgccgaagaattcttatgtgaaattcacataagcatgcccattactaaagacagtttgtataaagtaaccctaaatgtttattgaggaacctacagcttcaactgacttacgtgcagatatgtaccaggagaacatcattttagcttgggcgtctttacttggggttttcagaggatccaggaacctcactgtatgcaaagtcttgtggatgtacctgaatgtttttggaggcaggtcacatagtttctgaaagtgttctcttattttcctcaaatgtaggtaaccattgttacaagttatttaacaggagaatagtaacaatgtctaacttatgctaatgattttgtgtgctgagctcccattaattaaaatgtcttcagaaaaaaaaaaaaaaaaa

SEQ ID NO: 20 - DNA, 19 bp, Artificial Sequence
  Description of Artificial Sequence: Synthetic primer
ccaaccgcgagaagatgac

SEQ ID NO: 21 - DNA, 20 bp, Artificial Sequence
  Description of Artificial Sequence: Synthetic primer
tagcacagcctggatagcaa

SEQ ID NO: 22 - DNA, 20 bp, Artificial Sequence
  Description of Artificial Sequence: Synthetic primer
tgagaaaggaggctgcatca

SEQ ID NO: 23 - DNA, 19 bp, Artificial Sequence
  Description of Artificial Sequence: Synthetic primer
ctgctgcaactgctgaaca

SEQ ID NO: 24 - DNA, 23 bp, Artificial Sequence
  Description of Artificial Sequence: Synthetic primer
gcctcttccagaaactaggagaa

SEQ ID NO: 25 - DNA, 22 bp, Artificial Sequence
  Description of Artificial Sequence: Synthetic primer
ggggctttctttgtgtaagcaa

SEQ ID NO: 26 - DNA, 20 bp, Artificial Sequence
  Description of Artificial Sequence: Synthetic primer
gacagctgccaggatcctaa

SEQ ID NO: 27 - DNA, 22 bp, Artificial Sequence
  Description of Artificial Sequence: Synthetic primer
gtctggcacatgtttgtctaca

SEQ ID NO: 28 - DNA, 18 bp, Artificial Sequence
  Description of Artificial Sequence: Synthetic primer
aagtgcgccacaagcaaa

SEQ ID NO: 29 - DNA, 19 bp, Artificial Sequence
  Description of Artificial Sequence: Synthetic primer
tgccttatggcgagttcca

SEQ ID NO: 30 - DNA, 20 bp, Artificial Sequence
  Description of Artificial Sequence: Synthetic primer
cagcggcagctgattgttaa

SEQ ID NO: 31 - DNA, 23 bp, Artificial Sequence
  Description of Artificial Sequence: Synthetic primer
cagagagatcacccttcaagtca

SEQ ID NO: 32 - DNA, 20 bp, Artificial Sequence
  Description of Artificial Sequence: Synthetic primer
acccagatgactcccacaaa

SEQ ID NO: 33 - DNA, 20 bp, Artificial Sequence
  Description of Artificial Sequence: Synthetic primer
caaggattggctgctgctta

SEQ ID NO: 34 - DNA, 17 bp, Artificial Sequence
  Description of Artificial Sequence: Synthetic primer
aaggccgtggtcctgac

SEQ ID NO: 35 - DNA, 20 bp, Artificial Sequence
  Description of Artificial Sequence: Synthetic primer
tcagctggctgaagtagtcc

SEQ ID NO: 36 - DNA, 19 bp, Artificial Sequence
  Description of Artificial Sequence: Synthetic primer
gcaaggtggcagaagtcaa

SEQ ID NO: 37 - DNA, 19 bp, Artificial Sequence
  Description of Artificial Sequence: Synthetic primer
atggccagagatgcttcca

SEQ ID NO: 38 - DNA, 20 bp, Artificial Sequence
  Description of Artificial Sequence: Synthetic primer
gcgcctttcttcatcatcca

SEQ ID NO: 39 - DNA, 22 bp, Artificial Sequence
  Description of Artificial Sequence: Synthetic primer
gatggtgatggtagggttttcc

SEQ ID NO: 40 - DNA, 20 bp, Artificial Sequence
  Description of Artificial Sequence: Synthetic primer
tcctggaactgaagcactca

SEQ ID NO: 41 - DNA, 20 bp, Artificial Sequence
  Description of Artificial Sequence: Synthetic primer
gcagcacaagaatgggtaca

SEQ ID NO: 42 - DNA, 20 bp, Artificial Sequence
  Description of Artificial Sequence: Synthetic primer
ccccttcctggctctcagta

SEQ ID NO: 43 - DNA, 18 bp, Artificial Sequence
  Description of Artificial Sequence: Synthetic primer
ggtctgggctgctctcca

SEQ ID NO: 44 - DNA, 19 bp, Artificial Sequence
  Description of Artificial Sequence: Synthetic primer
ggacagtgaccctcaacca

SEQ ID NO: 45 - DNA, 22 bp, Artificial Sequence
  Description of Artificial Sequence: Synthetic primer
cagcagggcaaatctcttgtta

SEQ ID NO: 46 - DNA, 20 bp, Artificial Sequence
  Description of Artificial Sequence: Synthetic primer
tggaaaggtggtgtggaaac

SEQ ID NO: 47 - DNA, 19 bp, Artificial Sequence
  Description of Artificial Sequence: Synthetic primer
gtcagctggtggttgctaa

SEQ ID NO: 48 - DNA, 21 bp, Artificial Sequence
  Description of Artificial Sequence: Synthetic primer
tgatgtcagtgctgctactcc

SEQ ID NO: 49 - DNA, 23 bp, Artificial Sequence
  Description of Artificial Sequence: Synthetic primer
ctgtgtatccaagacagcagtca

SEQ ID NO: 50 - DNA, 20 bp, Artificial Sequence
  Description of Artificial Sequence: Synthetic primer
ctcagttcaggcttcctaca

SEQ ID NO: 51 - DNA, 20 bp, Artificial Sequence
  Description of Artificial Sequence: Synthetic primer
tcttttggcacaaggcttac

SEQ ID NO: 52 - DNA, 22 bp, Artificial Sequence
  Description of Artificial Sequence: Synthetic primer
cacaatagaaccttcagcagac

SEQ ID NO: 53 - DNA, 26 bp, Artificial Sequence
  Description of Artificial Sequence: Synthetic primer
gaaaagtgtcttcatgtatccagtta

SEQ ID NO: 54 - DNA, 20 bp, Artificial Sequence
  Description of Artificial Sequence: Synthetic primer
attccagcttcaacccctca

SEQ ID NO: 55 - DNA, 20 bp, Artificial Sequence
  Description of Artificial Sequence: Synthetic primer
atgactaggtgcctgggaac

SEQ ID NO: 56 - DNA, 20 bp, Artificial Sequence
  Description of Artificial Sequence: Synthetic primer
ccaactaatgccaccaccaa

SEQ ID NO: 57 - DNA, 20 bp, Artificial Sequence
  Description of Artificial Sequence: Synthetic primer
cgaagagactggctgttgac

SEQ ID NO: 58 - DNA, 21 bp, Artificial Sequence
  Description of Artificial Sequence: Synthetic primer
ccccttgcctacaagaagcta

SEQ ID NO: 59 - DNA, 17 bp, Artificial Sequence
  Description of Artificial Sequence: Synthetic primer
tcccgttgggccaatcc

SEQ ID NO: 60 - DNA, 20 bp, Artificial Sequence
  Description of Artificial Sequence: Synthetic primer
agcaagaacgccaaggacaa

SEQ ID NO: 61 - DNA, 20 bp, Artificial Sequence
  Description of Artificial Sequence: Synthetic primer
cggccacgattctcttccaa

SEQ ID NO: 62 - DNA, 20 bp, Artificial Sequence
  Description of Artificial Sequence: Synthetic primer
agattgcatgtcccctggaa

SEQ ID NO: 63 - DNA, 20 bp, Artificial Sequence
  Description of Artificial Sequence: Synthetic primer
gggtgggttccagaaggtta

SEQ ID NO: 64 - DNA, 20 bp, Artificial Sequence
  Description of Artificial Sequence: Synthetic primer
tatgcctgccacaccactaa

SEQ ID NO: 65 - DNA, 23 bp, Artificial Sequence
  Description of Artificial Sequence: Synthetic primer
gccaggagaacttccttgtacta

SEQ ID NO: 66 - DNA, 18 bp, Artificial Sequence
  Description of Artificial Sequence: Synthetic primer
tcaaccgccctgaacaca

SEQ ID NO: 67 - DNA, 21 bp, Artificial Sequence
  Description of Artificial Sequence: Synthetic primer
acaccgacaatgtgaccagaa

SEQ ID NO: 68 - DNA, 18 bp, Artificial Sequence
  Description of Artificial Sequence: Synthetic primer
agccttccaagcccatcc

SEQ ID NO: 69 - DNA, 20 bp, Artificial Sequence
  Description of Artificial Sequence: Synthetic primer
tgcggattgagaagccttta

SEQ ID NO: 70 - DNA, 20 bp, Artificial Sequence
  Description of Artificial Sequence: Synthetic primer
cgtggtcaggatggctagta

SEQ ID NO: 71 - DNA, 20 bp, Artificial Sequence
  Description of Artificial Sequence: Synthetic primer
ccaatcggcagcaatgtcta

SEQ ID NO: 72 - DNA, 21 bp, Artificial Sequence
  Description of Artificial Sequence: Synthetic primer
gtcctctgtgaaggggtcaaa

SEQ ID NO: 73 - DNA, 25 bp, Artificial Sequence
  Description of Artificial Sequence: Synthetic primer
tcttcaggcaagttagagttggtta

SEQ ID NO: 74 - DNA, 20 bp, Artificial Sequence
  Description of Artificial Sequence: Synthetic primer
tgacaacccagagctcatcc

SEQ ID NO: 75 - DNA, 20 bp, Artificial Sequence
  Description of Artificial Sequence: Synthetic primer
ggacgccatgttgtttggaa

SEQ ID NO: 76 - DNA, 21 bp, Artificial Sequence
  Description of Artificial Sequence: Synthetic primer
cgtccaggtgtcagaggatta

SEQ ID NO: 77 - DNA, 21 bp, Artificial Sequence
  Description of Artificial Sequence: Synthetic primer
accttgttctccaggataccc

SEQ ID NO: 78 - DNA, 20 bp, Artificial Sequence
  Description of Artificial Sequence: Synthetic primer
tgaagtggctggttacatcc

SEQ ID NO: 79 - DNA, 20 bp, Artificial Sequence
  Description of Artificial Sequence: Synthetic primer
agaggctggtcatagggtaa

SEQ ID NO: 80 - DNA, 20 bp, Artificial Sequence
  Description of Artificial Sequence: Synthetic primer
gtcttgaccagcctctctca

SEQ ID NO: 81 - DNA, 20 bp, Artificial Sequence
  Description of Artificial Sequence: Synthetic primer
acggtgctttgagggataca

SEQ ID NO: 82 - DNA, 20 bp, Artificial Sequence
  Description of Artificial Sequence: Synthetic primer
acaagagaccggctctagga

SEQ ID NO: 83 - DNA, 20 bp, Artificial Sequence
  Description of Artificial Sequence: Synthetic primer
ttgccactaggtgagctgtc

SEQ ID NO: 84 - DNA, 21 bp, Artificial Sequence
  Description of Artificial Sequence: Synthetic primer
cgttccgttatccaggctttt

SEQ ID NO: 85 - DNA, 21 bp, Artificial Sequence
  Description of Artificial Sequence: Synthetic primer
actcctggtaggtgtcaatgg

SEQ ID NO: 86 - DNA, 21 bp, Artificial Sequence
  Description of Artificial Sequence: Synthetic primer
ttagagctgctccacatctcc

SEQ ID NO: 87 - DNA, 21 bp, Artificial Sequence
  Description of Artificial Sequence: Synthetic primer
accaggttgttggtgaaggta

SEQ ID NO: 88 - DNA, 20 bp, Artificial Sequence
  Description of Artificial Sequence: Synthetic primer
tccatcaccaagagggtgaa

SEQ ID NO: 89 - DNA, 20 bp, Artificial Sequence
  Description of Artificial Sequence: Synthetic primer
caggatgctttccccaaaca

SEQ ID NO: 90 - DNA, 20 bp, Artificial Sequence
  Description of Artificial Sequence: Synthetic primer
acgtgcattgtgctctctca

SEQ ID NO: 91 - DNA, 22 bp, Artificial Sequence
  Description of Artificial Sequence: Synthetic primer
cagcactgatttggtcatctcc

SEQ ID NO: 92 - DNA, 19 bp, Artificial Sequence
  Description of Artificial Sequence: Synthetic primer
tgggcaccaaagaaggtta

SEQ ID NO: 93 - DNA, 20 bp, Artificial Sequence
  Description of Artificial Sequence: Synthetic primer
ttcctgtgcagagtaaacca

SEQ ID NO: 94 - DNA, 20 bp, Artificial Sequence
  Description of Artificial Sequence: Synthetic primer
atctctacgcccaccagtcc

SEQ ID NO: 95 - DNA, 20 bp, Artificial Sequence
  Description of Artificial Sequence: Synthetic primer
agcgagtccgagtcatccaa

SEQ ID NO: 96 - DNA, 20 bp, Artificial Sequence
  Description of Artificial Sequence: Synthetic primer
gacgaaagcttggctccaaa

SEQ ID NO: 97 - DNA, 20 bp, Artificial Sequence
  Description of Artificial Sequence: Synthetic primer
gttccatagcgacgttctcc

SEQ ID NO: 98 - DNA, 23 bp, Artificial Sequence
  Description of Artificial Sequence: Synthetic primer
tgggataaaagctctgctcttca

SEQ ID NO: 99 - DNA, 20 bp, Artificial Sequence
  Description of Artificial Sequence: Synthetic primer
tgttcgccggcagaatacta

SEQ ID NO: 100 - DNA, 21 bp, Artificial Sequence
  Description of Artificial Sequence: Synthetic primer
acaaggccaagaattccctca

SEQ ID NO: 101 - DNA, 19 bp, Artificial Sequence
  Description of Artificial Sequence: Synthetic primer
tgccggggcttcttaaaca

SEQ ID NO: 102 - DNA, 18 bp, Artificial Sequence
  Description of Artificial Sequence: Synthetic primer
ttcgtccccagccaacaa

SEQ ID NO: 103 - DNA, 20 bp, Artificial Sequence
  Description of Artificial Sequence: Synthetic primer
tggcttcccgttcactatcc

SEQ ID NO: 104 - DNA, 21 bp, Artificial Sequence
  Description of Artificial Sequence: Synthetic primer
gcagtgactttctcagcaaca

SEQ ID NO: 105 - DNA, 20 bp, Artificial Sequence
  Description of Artificial Sequence: Synthetic primer
ttgggacagcttggatcaca

SEQ ID NO: 106 - DNA, 17 bp, Artificial Sequence
  Description of Artificial Sequence: Synthetic primer
ctctgccgtcgcagcaa

SEQ ID NO: 107 - DNA, 20 bp, Artificial Sequence
  Description of Artificial Sequence: Synthetic primer
tggattagcccgttgcagac

SEQ ID NO: 108 - DNA, 21 bp, Artificial Sequence
  Description of Artificial Sequence: Synthetic primer
gccggagcaaaacttaggaaa

SEQ ID NO: 109 - DNA, 20 bp, Artificial Sequence
  Description of Artificial Sequence: Synthetic primer
aggcggagttcacaccaata

SEQ ID NO: 110 - DNA, 20 bp, Artificial Sequence
  Description of Artificial Sequence: Synthetic primer
gccaagctctggaggaagaa

SEQ ID NO: 111 - DNA, 22 bp, Artificial Sequence
  Description of Artificial Sequence: Synthetic primer
gagaagaacaggccgatggtta

SEQ ID NO: 112 - DNA, 17 bp, Artificial Sequence
  Description of Artificial Sequence: Synthetic primer
atcctggtgctgctgac

SEQ ID NO: 113 - DNA, 19 bp, Artificial Sequence
  Description of Artificial Sequence: Synthetic primer
ggccagatcttctgcttca

SEQ ID NO: 114 - DNA, 20 bp, Artificial Sequence
  Description of Artificial Sequence: Synthetic primer
agttcagaagagcccgagac

SEQ ID NO: 115 - DNA, 21 bp, Artificial Sequence
  Description of Artificial Sequence: Synthetic primer
gcgctgtcttttggtgaaaac

SEQ ID NO: 116 - DNA, 22 bp, Artificial Sequence
  Description of Artificial Sequence: Synthetic primer
taccgggagaactacgtatcca

SEQ ID NO: 117 - DNA, 17 bp, Artificial Sequence
  Description of Artificial Sequence: Synthetic primer
atgcgccggttctggaa

SEQ ID NO: 118 - DNA, 20 bp, Artificial Sequence
  Description of Artificial Sequence: Synthetic primer
aggaatgtgagctggagaca

SEQ ID NO: 119 - DNA, 21 bp, Artificial Sequence
  Description of Artificial Sequence: Synthetic primer
ttgtcaccttccaactgaacc

SEQ ID NO: 120 - DNA, 20 bp, Artificial Sequence
  Description of Artificial Sequence: Synthetic primer
gctacctggaagctgaccaa

SEQ ID NO: 121 - DNA, 19 bp, Artificial Sequence
  Description of Artificial Sequence: Synthetic primer
ccacctgcctagtggcaaa

SEQ ID NO: 122 - DNA, 20 bp, Artificial Sequence
  Description of Artificial Sequence: Synthetic primer
ggaaaggggtggatgtgtca

SEQ ID NO: 123 - DNA, 22 bp, Artificial Sequence
  Description of Artificial Sequence: Synthetic primer
cacccaggatgtccttgttcta

SEQ ID NO: 124 - DNA, 24 bp, Artificial Sequence
  Description of Artificial Sequence: Synthetic primer
atgttagagctcagttggttgata

SEQ ID NO: 125 - DNA, 20 bp, Artificial Sequence
  Description of Artificial Sequence: Synthetic primer
tactgcatgaccctcgacaa

SEQ ID NO: 126 - DNA, 20 bp, Artificial Sequence
  Description of Artificial Sequence: Synthetic primer
atattgtcgcaccccatgca

SEQ ID NO: 127 - DNA, 26 bp, Artificial Sequence
  Description of Artificial Sequence: Synthetic primer
acctcctttcctgataatttcctcac

SEQ ID NO: 128 - DNA, 20 bp, Artificial Sequence
  Description of Artificial Sequence: Synthetic primer
gccagcagcactttgagtta

SEQ ID NO: 129 - DNA, 20 bp, Artificial Sequence
  Description of Artificial Sequence: Synthetic primer
tgagtcaacacggagctgta

SEQ ID NO: 130 - DNA, 20 bp, Artificial Sequence
  Description of Artificial Sequence: Synthetic primer
gaaacccagccagaaagcaa

SEQ ID NO: 131 - DNA, 20 bp, Artificial Sequence
  Description of Artificial Sequence: Synthetic primer
aggtggtggtgtcagacaaa

SEQ ID NO: 132 - DNA, 23 bp, Artificial Sequence
  Description of Artificial Sequence: Synthetic primer
cctctgccctccacttaatgtta

SEQ ID NO: 133 - DNA, 22 bp, Artificial Sequence
  Description of Artificial Sequence: Synthetic primer
cagctatagagccttccaccaa

SEQ ID NO: 134 - DNA, 20 bp, Artificial Sequence
  Description of Artificial Sequence: Synthetic primer
ccggacctgagcgtcatgta

SEQ ID NO: 135 - DNA, 18 bp, Artificial Sequence
  Description of Artificial Sequence: Synthetic primer
gcacaccacgtgctcaca

SEQ ID NO: 136 - DNA, 21 bp, Artificial Sequence
  Description of Artificial Sequence: Synthetic primer
gaacgggaagcttgtcatcaa

SEQ ID NO: 137 - DNA, 20 bp, Artificial Sequence
  Description of Artificial Sequence: Synthetic primer
atcgccccacttgattttgg

SEQ ID NO: 138 - DNA, 21 bp, Artificial Sequence
  Description of Artificial Sequence: Synthetic primer
tcagtttggaaacctgcagaa

SEQ ID NO: 139 - DNA, 20 bp, Artificial Sequence
  Description of Artificial Sequence: Synthetic primer
gctgcccatagctctttgaa

SEQ ID NO: 140 - DNA, 16 bp, Artificial Sequence
  Description of Artificial Sequence: Synthetic primer
cccgtcgcctgtacca

SEQ ID NO: 141 - DNA, 24 bp, Artificial Sequence
  Description of Artificial Sequence: Synthetic primer
tgttggaatagactctgagaagca

SEQ ID NO: 142 - DNA, 21 bp, Artificial Sequence
  Description of Artificial Sequence: Synthetic primer
cggctacgacctgaaactcta

SEQ ID NO: 143 - DNA, 22 bp, Artificial Sequence
  Description of Artificial Sequence: Synthetic primer
tgagtgaggtgttgatgaacca

SEQ ID NO: 144 - DNA, 21 bp, Artificial Sequence
  Description of Artificial Sequence: Synthetic primer
ccagaggcagtgcaaacataa

SEQ ID NO: 145 - DNA, 20 bp, Artificial Sequence
  Description of Artificial Sequence: Synthetic primer
agaaattgggtccggggtta

SEQ ID NO: 146 - DNA, 19 bp, Artificial Sequence
  Description of Artificial Sequence: Synthetic primer
actccggacagcacataca

SEQ ID NO: 147 - DNA, 20 bp, Artificial Sequence
  Description of Artificial Sequence: Synthetic primer
ccaactgaagcactccgaaa

SEQ ID NO: 148 - DNA, 20 bp, Artificial Sequence
  Description of Artificial Sequence: Synthetic primer
aagacctggcaacggatgac

SEQ ID NO: 149 - DNA, 24 bp, Artificial Sequence
  Description of Artificial Sequence: Synthetic primer
ttgagaatcctttccaacccagac

SEQ ID NO: 150 - DNA, 21 bp, Artificial Sequence
  Description of Artificial Sequence: Synthetic primer
acaacttgtccatcgtttcac

SEQ ID NO: 151 - DNA, 18 bp, Artificial Sequence
  Description of Artificial Sequence: Synthetic primer
accagccatcacacacaa

SEQ ID NO: 152 - DNA, 19 bp, Artificial Sequence
  Description of Artificial Sequence: Synthetic primer
agaactgaacagcgcaaca

SEQ ID NO: 153 - DNA, 20 bp, Artificial Sequence
  Description of Artificial Sequence: Synthetic primer
gctgggtattcaccatggaa

SEQ ID NO: 154 - DNA, 20 bp, Artificial Sequence
  Description of Artificial Sequence: Synthetic primer
ggtgaccgttttggcaatcc

SEQ ID NO: 155 - DNA, 19 bp, Artificial Sequence
  Description of Artificial Sequence: Synthetic primer
cactggccactccagtcac

SEQ ID NO: 156 - DNA, 19 bp, Artificial Sequence
  Description of Artificial Sequence: Synthetic primer
gcctggcgcattacaacaa

SEQ ID NO: 157 - DNA, 20 bp, Artificial Sequence
  Description of Artificial Sequence: Synthetic primer
caattccccgggtagcagta

SEQ ID NO: 158 - DNA, 22 bp, Artificial Sequence
  Description of Artificial Sequence: Synthetic primer
cggcaaagctgaaggagaagta

SEQ ID NO: 159 - DNA, 20 bp, Artificial Sequence
  Description of Artificial Sequence: Synthetic primer
caggaccctttgcaccatca

SEQ ID NO: 160 - DNA, 21 bp, Artificial Sequence
  Description of Artificial Sequence: Synthetic primer
acacagtgctaggtgcagtta

SEQ ID NO: 161 - DNA, 21 bp, Artificial Sequence
  Description of Artificial Sequence: Synthetic primer
tccatactcccagcctttcac

SEQ ID NO: 162 - DNA, 19 bp, Artificial Sequence
  Description of Artificial Sequence: Synthetic primer
aagttcatccggcccttca

SEQ ID NO: 163 - DNA, 20 bp, Artificial Sequence
  Description of Artificial Sequence: Synthetic primer
ggtgtcttcatccacctcca

SEQ ID NO: 164 - DNA, 23 bp, Artificial Sequence
  Description of Artificial Sequence: Synthetic primer
tggacgtaagggactcaaaatcc

SEQ ID NO: 165 - DNA, 17 bp, Artificial Sequence
  Description of Artificial Sequence: Synthetic primer
cccaggcctgcgttaca

SEQ ID NO: 166 - DNA, 20 bp, Artificial Sequence
  Description of Artificial Sequence: Synthetic primer
tgtgccttacgacccatgta

SEQ ID NO: 167 - DNA, 20 bp, Artificial Sequence
  Description of Artificial Sequence: Synthetic primer
gttgttcagggcctcgttta

SEQ ID NO: 168 - DNA, 23 bp, Artificial Sequence
  Description of Artificial Sequence: Synthetic primer
gcaagaaggtggcattgtttcta

SEQ ID NO: 169 - DNA, 20 bp, Artificial Sequence
  Description of Artificial Sequence: Synthetic primer
tctggggaaagtgaggcaaa

SEQ ID NO: 170 - DNA, 22 bp, Artificial Sequence
  Description of Artificial Sequence: Synthetic primer
agagaagagaaggctggtgaac

SEQ ID NO: 171 - DNA, 20 bp, Artificial Sequence
  Description of Artificial Sequence: Synthetic primer
tccaggttgtcaggagcaaa

SEQ ID NO: 172 - DNA, 22 bp, Artificial Sequence
  Description of Artificial Sequence: Synthetic primer
tcccatctcaaagcccattaca

SEQ ID NO: 173 - DNA, 18 bp, Artificial Sequence
  Description of Artificial Sequence: Synthetic primer
ctcgtctgagcgggagaa

SEQ ID NO: 174 - DNA, 21 bp, Artificial Sequence
  Description of Artificial Sequence: Synthetic primer
ctggcaggactgtgagtacaa

SEQ ID NO: 175 - DNA, 22 bp, Artificial Sequence
  Description of Artificial Sequence: Synthetic primer
atttcgtactgctcctcttccc

SEQ ID NO: 176 - DNA, 21 bp, Artificial Sequence
  Description of Artificial Sequence: Synthetic primer
tgaccgacgagatcaacttcc

SEQ ID NO: 177 - DNA, 19 bp, Artificial Sequence
  Description of Artificial Sequence: Synthetic primer
tgtgccttgacctcagcaa

SEQ ID NO: 178 - DNA, 19 bp, Artificial Sequence
  Description of Artificial Sequence: Synthetic primer
tgaaggcattggggctgtg

SEQ ID NO: 179 - DNA, 18 bp, Artificial Sequence
  Description of Artificial Sequence: Synthetic primer
agcctgacacgcagaggt

SEQ ID NO: 180 - DNA, 20 bp, Artificial Sequence
  Description of Artificial Sequence: Synthetic primer
tgtgcatctatgtgcgtcac

SEQ ID NO: 181 - DNA, 22 bp, Artificial Sequence
  Description of Artificial Sequence: Synthetic primer
ggaatcgatgggcaaagttgta

SEQ ID NO: 182 - DNA, 20 bp, Artificial Sequence
  Description of Artificial Sequence: Synthetic primer
caaaagacgggcctcaccaa

SEQ ID NO: 183 - DNA, 20 bp, Artificial Sequence
  Description of Artificial Sequence: Synthetic primer
cgtaagaggttgcgcctgaa

SEQ ID NO: 184 - DNA, 18 bp, Artificial Sequence
  Description of Artificial Sequence: Synthetic primer
catcggtggaacgcacaa

SEQ ID NO: 185 - DNA, 20 bp, Artificial Sequence
  Description of Artificial Sequence: Synthetic primer
gggcacttccctcaaacaaa

SEQ ID NO: 186 - DNA, 20 bp, Artificial Sequence
  Description of Artificial Sequence: Synthetic primer
gccttggttggactggaaaa

SEQ ID NO: 187 - DNA, 22 bp, Artificial Sequence
  Description of Artificial Sequence: Synthetic primer
tttgaagagcaacatggggtac

SEQ ID NO: 188 - DNA, 20 bp, Artificial Sequence
  Description of Artificial Sequence: Synthetic primer
ctcccaggaaccgtacttca

SEQ ID NO: 189 - DNA, 22 bp, Artificial Sequence
  Description of Artificial Sequence: Synthetic primer
ctctgataaaagccacgtctcc

SEQ ID NO: 190 - DNA, 21 bp, Artificial Sequence
  Description of Artificial Sequence: Synthetic primer
catcaagatgtggcaggagta

SEQ ID NO: 191 - DNA, 23 bp, Artificial Sequence
  Description of Artificial Sequence: Synthetic primer
tgcagtaccatgacactgaaata

SEQ ID NO: 192 - DNA, 23 bp, Artificial Sequence
  Description of Artificial Sequence: Synthetic primer
gactccattcctttggtctttcc

SEQ ID NO: 193 - DNA, 20 bp, Artificial Sequence
  Description of Artificial Sequence: Synthetic primer
ccatggattcctcggagtca

SEQ ID NO: 194 - DNA, 20 bp, Artificial Sequence
  Description of Artificial Sequence: Synthetic primer
tggtctgatgggtggagacc

SEQ ID NO: 195 - DNA, 22 bp, Artificial Sequence
  Description of Artificial Sequence: Synthetic primer
tgagtttcggggattgccatac

SEQ ID NO: 196 - DNA, 22 bp, Artificial Sequence
  Description of Artificial Sequence: Synthetic primer
tctcacaatgggattctctcca

SEQ ID NO: 197 - DNA, 20 bp, Artificial Sequence
  Description of Artificial Sequence: Synthetic primer
caggcaagttcctgaagtcc

SEQ ID NO: 198 - DNA, 21 bp, Artificial Sequence
  Description of Artificial Sequence: Synthetic primer
tgccgaagaaacatggaccaa

SEQ ID NO: 199 - DNA, 20 bp, Artificial Sequence
  Description of Artificial Sequence: Synthetic primer
agccccaaagaatggccaaa

SEQ ID NO: 200 - DNA, 19 bp, Artificial Sequence
  Description of Artificial Sequence: Synthetic primer
agaaggccaaaccccagaa

SEQ ID NO: 201 - DNA, 19 bp, Artificial Sequence
  Description of Artificial Sequence: Synthetic primer
atgctgaggccttgtttgc

SEQ ID NO: 202 - DNA, 21 bp, Artificial Sequence
  Description of Artificial Sequence: Synthetic primer
gagagttgtccagtgatgtca

SEQ ID NO: 203 - DNA, 20 bp, Artificial Sequence
  Description of Artificial Sequence: Synthetic primer
gtcctgaacccaagtcatca

SEQ ID NO: 204 - DNA, 21 bp, Artificial Sequence
  Description of Artificial Sequence: Synthetic primer
catcggtacccagttcaggaa

SEQ ID NO: 205 - DNA, 19 bp, Artificial Sequence
  Description of Artificial Sequence: Synthetic primer
tgctgcatgctgaacacac

SEQ ID NO: 206 - DNA, 21 bp, Artificial Sequence
  Description of Artificial Sequence: Synthetic primer
tcctctccaacaccaaagtcc

SEQ ID NO: 207 - DNA, 19 bp, Artificial Sequence
  Description of Artificial Sequence: Synthetic primer
aggattccggcacagtcaa

SEQ ID NO: 208 - DNA, 19 bp, Artificial Sequence
  Description of Artificial Sequence: Synthetic primer
tggaagccacggtggataa

SEQ ID NO: 209 - DNA, 20 bp, Artificial Sequence
  Description of Artificial Sequence: Synthetic primer
tgtgcggatatgcttgttcc

SEQ ID NO: 210 - DNA, 19 bp, Artificial Sequence
  Description of Artificial Sequence: Synthetic primer
tctgctcccttccattccc

SEQ ID NO: 211 - DNA, 26 bp, Artificial Sequence
  Description of Artificial Sequence: Synthetic primer
gaattcttcattcccttgaactgaac

SEQ ID NO: 212 - DNA, 19 bp, Artificial Sequence
  Description of Artificial Sequence: Synthetic primer
cgcctcatgttctgctaca

SEQ ID NO: 213 - DNA, 20 bp, Artificial Sequence
  Description of Artificial Sequence: Synthetic primer
tagaagagtgcgttggtcac

SEQ ID NO: 214 - DNA, 19 bp, Artificial Sequence
  Description of Artificial Sequence: Synthetic primer
cgagccgaccatgtcttca

SEQ ID NO: 215 - DNA, 20 bp, Artificial Sequence
  Description of Artificial Sequence: Synthetic primer
aagctgaaggttcggagcaa

SEQ ID NO: 216 - DNA, 21 bp, Artificial Sequence
  Description of Artificial Sequence: Synthetic primer
ccaggctttccaaggttacca

SEQ ID NO: 217 - DNA, 18 bp, Artificial Sequence
  Description of Artificial Sequence: Synthetic primer
tggctttctgggcaagca

SEQ ID NO: 218 - DNA, 23 bp, Artificial Sequence
  Description of Artificial Sequence: Synthetic primer
actggatacattcaaaccctcca

SEQ ID NO: 219 - DNA, 20 bp, Artificial Sequence
  Description of Artificial Sequence: Synthetic primer
tggtgcacagactggtgtta

SEQ ID NO: 220 - DNA, 23 bp, Artificial Sequence
  Description of Artificial Sequence: Synthetic primer
gtactgtggcgatggcattatac

SEQ ID NO: 221 - DNA, 20 bp, Artificial Sequence
  Description of Artificial Sequence: Synthetic primer
agaaaagggagcagccatca

SEQ ID NO: 222 - DNA, 20 bp, Artificial Sequence
  Description of Artificial Sequence: Synthetic primer
acagtggaagcctgggttaa

SEQ ID NO: 223 - DNA, 21 bp, Artificial Sequence
  Description of Artificial Sequence: Synthetic primer
acagtgtgggagcagttatca

SEQ ID NO: 224 - DNA, 20 bp, Artificial Sequence
  Description of Artificial Sequence: Synthetic primer
ctggcatccagttgacgaaa

SEQ ID NO: 225 - DNA, 20 bp, Artificial Sequence
  Description of Artificial Sequence: Synthetic primer
catcagggcctagcaggtaa

SEQ ID NO: 226 - DNA, 20 bp, Artificial Sequence
  Description of Artificial Sequence: Synthetic primer
gtgcagcactaccacatgaa

SEQ ID NO: 227 - DNA, 20 bp, Artificial Sequence
  Description of Artificial Sequence: Synthetic primer
tatacgagcccgtcttctcc

SEQ ID NO: 228 - DNA, 22 bp, Artificial Sequence
  Description of Artificial Sequence: Synthetic primer
gccagctgctatatcacacaaa

SEQ ID NO: 229 - DNA, 20 bp, Artificial Sequence
  Description of Artificial Sequence: Synthetic primer
aaacccagggctacttccaa

SEQ ID NO: 230 - DNA, 23 bp, Artificial Sequence
  Description of Artificial Sequence: Synthetic primer
gccacatttcaaaggaaactgac

SEQ ID NO: 231 - DNA, 20 bp, Artificial Sequence
  Description of Artificial Sequence: Synthetic primer
tccctgcagccaatcagata

SEQ ID NO: 232 - DNA, 20 bp, Artificial Sequence
  Description of Artificial Sequence: Synthetic primer
ccaccaagaagccactttcc

SEQ ID NO: 233 - DNA, 20 bp, Artificial Sequence
  Description of Artificial Sequence: Synthetic primer
taccagcaatgccagggtta

SEQ ID NO: 234 - DNA, 20 bp, Artificial Sequence
  Description of Artificial Sequence: Synthetic primer
agaaactgcgtccgttttcc

SEQ ID NO: 235 - DNA, 23 bp, Artificial Sequence
  Description of Artificial Sequence: Synthetic primer
ggagtcagatgtccttgggataa

SEQ ID NO: 236 - DNA, 22 bp, Artificial Sequence
  Description of Artificial Sequence: Synthetic primer
cggatcaaactgggatttaccc

SEQ ID NO: 237 - DNA, 20 bp, Artificial Sequence
  Description of Artificial Sequence: Synthetic primer
cgagaacacgttgccataca

SEQ ID NO: 238 - DNA, 19 bp, Artificial Sequence
  Description of Artificial Sequence: Synthetic primer
tctggcttcctccaccaaa

SEQ ID NO: 239 - DNA, 20 bp, Artificial Sequence
  Description of Artificial Sequence: Synthetic primer
cagcggagttcagcatacaa

SEQ ID NO: 240 - DNA, 18 bp, Artificial Sequence
  Description of Artificial Sequence: Synthetic primer
gttcggctcctggctgat

SEQ ID NO: 241 - DNA, 22 bp, Artificial Sequence
  Description of Artificial Sequence: Synthetic primer
caaagatggacaccagcgaatc

SEQ ID NO: 242 - DNA, 20 bp, Artificial Sequence
  Description of Artificial Sequence: Synthetic primer
ggggcagtttctgctcttca

SEQ ID NO: 243 - DNA, 21 bp, Artificial Sequence
  Description of Artificial Sequence: Synthetic primer
tcatcctcaggcagcgtctta

SEQ ID NO: 244 - DNA, 22 bp, Artificial Sequence
  Description of Artificial Sequence: Synthetic primer
gcaggatcctacaccttacaca

SEQ ID NO: 245 - DNA, 20 bp, Artificial Sequence
  Description of Artificial Sequence: Synthetic primer
tgctggagatggagggctta

SEQ ID NO: 246 - DNA, 18 bp, Artificial Sequence
  Description of Artificial Sequence: Synthetic primer
ctggcgaggaaagctcca

SEQ ID NO: 247 - DNA, 23 bp, Artificial Sequence
  Description of Artificial Sequence: Synthetic primer
cagaaatgacatcacagctgcta

SEQ ID NO: 248 - DNA, 21 bp, Artificial Sequence
  Description of Artificial Sequence: Synthetic primer
ctccccagcatttacccttca

SEQ ID NO: 249 - DNA, 19 bp, Artificial Sequence
  Description of Artificial Sequence: Synthetic primer
ggttagactcggcgaagca

SEQ ID NO: 250 - DNA, 20 bp, Artificial Sequence
  Description of Artificial Sequence: Synthetic primer
acccagtcaccctgaatgtc

SEQ ID NO: 251 - DNA, 23 bp, Artificial Sequence
  Description of Artificial Sequence: Synthetic primer
gcaggacaagtagaggttttgtc

SEQ ID NO: 252 - DNA, 18 bp, Artificial Sequence
  Description of Artificial Sequence: Synthetic primer
gtcggtctgctggtctcc

SEQ ID NO: 253 - DNA, 20 bp, Artificial Sequence
  Description of Artificial Sequence: Synthetic primer
tgtgtcttgcagtgctcaac

SEQ ID NO: 254 - DNA, 20 bp, Artificial Sequence
  Description of Artificial Sequence: Synthetic primer
aggcacagatatgggacaca

SEQ ID NO: 255 - DNA, 20 bp, Artificial Sequence
  Description of Artificial Sequence: Synthetic primer
ataaggcacctacagctcca

SEQ ID NO: 256 - DNA, 20 bp, Artificial Sequence
  Description of Artificial Sequence: Synthetic primer
accagatcagagggaagtca

SEQ ID NO: 257 - DNA, 20 bp, Artificial Sequence
  Description of Artificial Sequence: Synthetic primer
cagttgctgcacttgtttca

SEQ ID NO: 258 - DNA, 20 bp, Artificial Sequence
  Description of Artificial Sequence: Synthetic primer
ggaagcaggatggatgaaca

SEQ ID NO: 259 - DNA, 21 bp, Artificial Sequence
  Description of Artificial Sequence: Synthetic primer
ctcgggtatggaatgtagtcc

SEQ ID NO: 260 - DNA, 20 bp, Artificial Sequence
  Description of Artificial Sequence: Synthetic primer
tgaagacacccgctccagta

SEQ ID NO: 261 - DNA, 21 bp, Artificial Sequence
  Description of Artificial Sequence: Synthetic primer
ccccatttcactgcctcttca

SEQ ID NO: 262 - DNA, 20 bp, Artificial Sequence
  Description of Artificial Sequence: Synthetic primer
tgggaaggtggtcatcacac

SEQ ID NO: 263 - DNA, 18 bp, Artificial Sequence
  Description of Artificial Sequence: Synthetic primer
cagcacccgctgagatca

SEQ ID NO: 264 - DNA, 20 bp, Artificial Sequence
  Description of Artificial Sequence: Synthetic primer
gccaagatcccatctctcca

SEQ ID NO: 265 - DNA, 20 bp, Artificial Sequence
  Description of Artificial Sequence: Synthetic primer
aggcacttcagctcaggaaa

SEQ ID NO: 266 - DNA, 20 bp, Artificial Sequence
  Description of Artificial Sequence: Synthetic primer
ctggctgtgggtgtggtact

SEQ ID NO: 267 - DNA, 19 bp, Artificial Sequence
  Description of Artificial Sequence: Synthetic primer
cgctccactccctctaggc

SEQ ID NO: 268 - DNA, 21 bp, Artificial Sequence
  Description of Artificial Sequence: Synthetic primer
gctagagaccgagtgtcctca

SEQ ID NO: 269 - DNA, 22 bp, Artificial Sequence
  Description of Artificial Sequence: Synthetic primer
ccagaatgaggaactcctggaa

SEQ ID NO: 270 - DNA, 20 bp, Artificial Sequence
  Description of Artificial Sequence: Synthetic primer
tcaaagagctggtgcgaaaa

SEQ ID NO: 271 - DNA, 20 bp, Artificial Sequence
  Description of Artificial Sequence: Synthetic primer
atttgtgtccaggtcctcca

SEQ ID NO: 272 - DNA, 20 bp, Artificial Sequence
  Description of Artificial Sequence: Synthetic primer
gaaggagctaccaggcttcc

SEQ ID NO: 273 - DNA, 21 bp, Artificial Sequence
  Description of Artificial Sequence: Synthetic primer
agcaatttatccacggcatcc

SEQ ID NO: 274 - DNA, 20 bp, Artificial Sequence
  Description of Artificial Sequence: Synthetic primer
cttcgagaagtcttgcaacc

SEQ ID NO: 275 - DNA, 21 bp, Artificial Sequence
  Description of Artificial Sequence: Synthetic primer
gccagaataagagggaagcta

SEQ ID NO: 276 - DNA, 20 bp, Artificial Sequence
  Description of Artificial Sequence: Synthetic primer
tttgccaaagtggctgcaaa

SEQ ID NO: 277 - DNA, 20 bp, Artificial Sequence
  Description of Artificial Sequence: Synthetic primer
tttctgggcttgggttctcc

SEQ ID NO: 278 - DNA, 19 bp, Artificial Sequence
  Description of Artificial Sequence: Synthetic primer
tgcaccagtgggtgtcata

SEQ ID NO: 279 - DNA, 20 bp, Artificial Sequence
  Description of Artificial Sequence: Synthetic primer
gtggaactgaaggtgccaaa

SEQ ID NO: 280 - DNA, 22 bp, Artificial Sequence
  Description of Artificial Sequence: Synthetic primer
agaagtggaaccgcttactaca

SEQ ID NO: 281 - DNA, 20 bp, Artificial Sequence
  Description of Artificial Sequence: Synthetic primer
agtgtggctccaaggtcata

SEQ ID NO: 282 - DNA, 22 bp, Artificial Sequence
  Description of Artificial Sequence: Synthetic primer
gctgccatcgtgtatttctaca

SEQ ID NO: 283 - DNA, 20 bp, Artificial Sequence
  Description of Artificial Sequence: Synthetic primer
agacctcatccaccggaaaa

SEQ ID NO: 284 - DNA, 21 bp, Artificial Sequence
  Description of Artificial Sequence: Synthetic primer
gggagcacttggcacttttca

SEQ ID NO: 285 - DNA, 20 bp, Artificial Sequence
  Description of Artificial Sequence: Synthetic primer
gcaggatgtgccacagatca

SEQ ID NO: 286 - DNA, 22 bp, Artificial Sequence
  Description of Artificial Sequence: Synthetic primer
ggtccttcccatctacagtgaa

SEQ ID NO: 287 - DNA, 21 bp, Artificial Sequence
  Description of Artificial Sequence: Synthetic primer
agcatccccgtgatggaaata

SEQ ID NO: 288 - DNA, 18 bp, Artificial Sequence
  Description of Artificial Sequence: Synthetic primer
tgctgccgctcatcttca

SEQ ID NO: 289 - DNA, 20 bp, Artificial Sequence
  Description of Artificial Sequence: Synthetic primer
caaaggttgccttggcatca

SEQ ID NO: 290 - DNA, 19 bp, Artificial Sequence
  Description of Artificial Sequence: Synthetic primer
gacctggcgctccagttta

SEQ ID NO: 291 - DNA, 22 bp, Artificial Sequence
  Description of Artificial Sequence: Synthetic primer
cctctgtgaagcatctcagcta

SEQ ID NO: 292 - DNA, 21 bp, Artificial Sequence
  Description of Artificial Sequence: Synthetic primer
aagacggcttgatttcaggaa

SEQ ID NO: 293 - DNA, 20 bp, Artificial Sequence
  Description of Artificial Sequence: Synthetic primer
gcatcatccaatggtctcca

SEQ ID NO: 294 - DNA, 21 bp, Artificial Sequence
  Description of Artificial Sequence: Synthetic primer
tgttaagcaggacgactttcc

SEQ ID NO: 295 - DNA, 20 bp, Artificial Sequence
  Description of Artificial Sequence: Synthetic primer
cctttctggctgggcttaaa

SEQ ID NO: 296 - DNA, 18 bp, Artificial Sequence
  Description of Artificial Sequence: Synthetic primer
ggtgcctctgccttccaa

SEQ ID NO: 297 - DNA, 20 bp, Artificial Sequence
  Description of Artificial Sequence: Synthetic primer
ttgtgccagccatagtcaca

SEQ ID NO: 298 - DNA, 22 bp, Artificial Sequence
  Description of Artificial Sequence: Synthetic primer
agagtgaaggtgtgatgctgaa

SEQ ID NO: 299 - DNA, 20 bp, Artificial Sequence
  Description of Artificial Sequence: Synthetic primer
gcacggtttgtgacaggtac